European Patent Specification EP 3 277 321 B1, published August 14, 2024. Title: ANTIBODIES DIRECTED AGAINST T CELL IMMUNOGLOBULIN AND MUCIN PROTEIN 3 (TIM-3). Applicant: AnaptysBio, Inc. The sequence listing filed with the application follows.

SEQUENCE LISTING (340 sequences)

SEQ ID NO: 1 - protein, 121 aa, Artificial Sequence
  Synthetic Sequence
  MISC_FEATURE (23)..(23): Xaa1 is deleted or is alanine (Ala)
  MISC_FEATURE (25)..(25): Xaa2 is alanine (Ala), proline (Pro), aspartic acid (Asp), glycine (Gly), threonine (Thr), or valine (Val)
  MISC_FEATURE (29)..(31): the subsequence Xaa3 Xaa4 Xaa5 is deleted or is Thr-Phe-Ile
  MISC_FEATURE (35)..(35): Xaa6 is serine (Ser),  asparagine (Asn), arginine (Arg), or threonine (Thr)
  MISC_FEATURE (37)..(37): Xaa7 is aspartic acid (Asp) or alanine (Ala)
  MISC_FEATURE (39)..(39): Xaa8 is serine (Ser) or threonine (Thr)
  MISC_FEATURE (45)..(45): Xaa9 is proline (Pro) or leucine (Leu)
  MISC_FEATURE (50)..(50): Xaa10 is aspartic acid (Asp) or glutamic acid (Glu)
  MISC_FEATURE (54)..(54): Xaa11 is threonine (Thr) or alanine (Ala)
  MISC_FEATURE (57)..(57): Xaa12 is glycine (Gly) or serine (Ser)
  MISC_FEATURE (60)..(60): Xaa13 is serine (Ser), threonine (Thr), aspartic acid (Asp), glycine (Gly), asparagine (Asn), or lysine (Lys)
  MISC_FEATURE (92)..(92): Xaa14 is alanine (Ala) or valine (Val)
  MISC_FEATURE (101)..(101): Xaa15 is alanine (Ala) or threonine (Thr)
  MISC_FEATURE (103)..(106): the subsequence Xaa16 Xaa17 Xaa18 Xaa19 is deleted or is Pro-Tyr-Tyr-Ala
EVQLLESGGGLVQPGGSLRLSCXAXSGFXXXTFSXYXMXWVRQAXGKGLXWVSXISXGGXYTYYQDSVKGRFTISRDNSKNTLYLQMNSLRXEDTAVYYCXSXXXXMDYWGQGTTVTVSSA

SEQ ID NO: 2 - protein, 117 aa, Artificial Sequence
  Synthetic Sequence
EVQLLESGGGLVQPGGSLRLSCAASGFTFSSYDMSWVRQAPGKGLEWVSTISGGGSYTYYQDSVKGRFTISRDNSKNTLYLQMNSLRAEDTAVYYCASPYYAMDYWGQGTTVTVSSA

SEQ ID NO: 3 - protein, 113 aa, Artificial Sequence
  Synthetic Sequence
EVQLLESGGGLVQPGGSLRLSCAASGFTFSSYDMSWVRQAPGKGLEWVSTISGGGTYTYYQDSVKGRFTISRDNSKNTLYLQMNSLRAEDTAVYYCASMDYWGQGTTVTVSSA

SEQ ID NO: 4 - protein, 116 aa, Artificial Sequence
  Synthetic Sequence
EVQLLESGGGLVQPGGSLRLSCAASGFTFITFSSYDMSWVRQAPGKGLEWVSTISGGGSYTYYQDSVKGRFTISRDNSKNTLYLQMNSLRAEDTAVYYCASMDYWGQGTTVTVSSA

SEQ ID NO: 5 - protein, 113 aa, Artificial Sequence
  Synthetic Sequence
EVQLLESGGGLVQPGGSLRLSCAASGFTFSSYDMSWVRQAPGKGLEWVSTISSGGSYTYYQDSVKGRFTISRDNSKNTLYLQMNSLRAEDTAVYYCASMDYWGQGTTVTVSSA

SEQ ID NO: 6 - protein, 113 aa, Artificial Sequence
  Synthetic Sequence
EVQLLESGGGLVQPGGSLRLSCAASGFTFSSYDMSWVRQAPGKGLEWVSTISGGGSYTYYQDSVKGRFTISRDNSKNTLYLQMNSLRAEDTAVYYCTSMDYWGQGTTVTVSSA

SEQ ID NO: 7 - protein, 114 aa, Artificial Sequence
  Synthetic Sequence
EVQLLESGGGLVQPGGSLRLSCAAASGFTFSSYDMSWVRQAPGKGLEWVSTISGGGTYTYYQDSVKGRFTISRDNSKNTLYLQMNSLRAEDTAVYYCASMDYWGQGTTVTVSSA

SEQ ID NO: 8 - protein, 114 aa, Artificial Sequence
  Synthetic Sequence
EVQLLESGGGLVQPGGSLRLSCAAASGFTFSNYDMSWVRQAPGKGLEWVSTISGGGSYTYYQDSVKGRFTISRDNSKNTLYLQMNSLRAEDTAVYYCASMDYWGQGTTVTVSSA

SEQ ID NO: 9 - protein, 117 aa, Artificial Sequence
  Synthetic Sequence
EVQLLESGGGLVQPGGSLRLSCAAASGFTFITFSSYDMSWVRQAPGKGLEWVSTISGGGTYTYYQDSVKGRFTISRDNSKNTLYLQMNSLRAEDTAVYYCASMDYWGQGTTVTVSSA

SEQ ID NO: 10 - protein, 114 aa, Artificial Sequence
  Synthetic Sequence
EVQLLESGGGLVQPGGSLRLSCAAASGFTFSSYDMSWVRQAPGKGLEWVSTISGGGTYTYYQDSVKGRFTISRDNSKNTLYLQMNSLRAEDTAVYYCTSMDYWGQGTTVTVSSA

SEQ ID NO: 11 - protein, 114 aa, Artificial Sequence
  Synthetic Sequence
EVQLLESGGGLVQPGGSLRLSCAAASGFTFSSYDMSWVRQAPGKGLEWVSTISSGGTYTYYQDSVKGRFTISRDNSKNTLYLQMNSLRAEDTAVYYCASMDYWGQGTTVTVSSA

SEQ ID NO: 12 - protein, 114 aa, Artificial Sequence
  Synthetic Sequence
EVQLLESGGGLVQPGGSLRLSCAAPSGFTFSSYDMSWVRQAPGKGLEWVSTISGGGTYTYYQDSVKGRFTISRDNSKNTLYLQMNSLRAEDTAVYYCASMDYWGQGTTVTVSSA

SEQ ID NO: 13 - protein, 117 aa, Artificial Sequence
  Synthetic Sequence
EVQLLESGGGLVQPGGSLRLSCAAPSGFTFITFSSYDMSWVRQAPGKGLEWVSTISGGGTYTYYQDSVKGRFTISRDNSKNTLYLQMNSLRAEDTAVYYCASMDYWGQGTTVTVSSA

SEQ ID NO: 14 - protein, 113 aa, Artificial Sequence
  Synthetic Sequence
EVQLLESGGGLVQPGGSLRLSCAPSGFTFSSYDMSWVRQAPGKGLEWVSTISGGGTYTYYQDSVKGRFTISRDNSKNTLYLQMNSLRAEDTAVYYCASMDYWGQGTTVTVSSA

SEQ ID NO: 15 - protein, 114 aa, Artificial Sequence
  Synthetic Sequence
EVQLLESGGGLVQPGGSLRLSCAAASGFTFSRYDMSWVRQAPGKGLEWVSTISGGGTYTYYQDSVKGRFTISRDNSKNTLYLQMNSLRAEDTAVYYCASMDYWGQGTTVTVSSA

SEQ ID NO: 16 - protein, 113 aa, Artificial Sequence
  Synthetic Sequence
EVQLLESGGGLVQPGGSLRLSCADSGFTFSSYDMSWVRQAPGKGLEWVSTISGGGTYTYYQDSVKGRFTISRDNSKNTLYLQMNSLRAEDTAVYYCASMDYWGQGTTVTVSSA

SEQ ID NO: 17 - protein, 113 aa, Artificial Sequence
  Synthetic Sequence
EVQLLESGGGLVQPGGSLRLSCAGSGFTFSSYDMSWVRQAPGKGLEWVSTISGGGTYTYYQDSVKGRFTISRDNSKNTLYLQMNSLRAEDTAVYYCASMDYWGQGTTVTVSSA

SEQ ID NO: 18 - protein, 114 aa, Artificial Sequence
  Synthetic Sequence
EVQLLESGGGLVQPGGSLRLSCAATSGFTFSSYDMSWVRQAPGKGLEWVSTISGGGTYTYYQDSVKGRFTISRDNSKNTLYLQMNSLRAEDTAVYYCASMDYWGQGTTVTVSSA

SEQ ID NO: 19 - protein, 114 aa, Artificial Sequence
  Synthetic Sequence
EVQLLESGGGLVQPGGSLRLSCAAVSGFTFSSYDMSWVRQAPGKGLEWVSTISGGGTYTYYQDSVKGRFTISRDNSKNTLYLQMNSLRAEDTAVYYCASMDYWGQGTTVTVSSA

SEQ ID NO: 20 - protein, 114 aa, Artificial Sequence
  Synthetic Sequence
EVQLLESGGGLVQPGGSLRLSCAAASGFTFSSYDMSWVRQAPGKGLEWVSAISGGGTYTYYQDSVKGRFTISRDNSKNTLYLQMNSLRAEDTAVYYCASMDYWGQGTTVTVSSA

SEQ ID NO: 21 - protein, 114 aa, Artificial Sequence
  Synthetic Sequence
EVQLLESGGGLVQPGGSLRLSCAAASGFTFSSYAMSWVRQAPGKGLEWVSTISGGGTYTYYQDSVKGRFTISRDNSKNTLYLQMNSLRAEDTAVYYCASMDYWGQGTTVTVSSA

SEQ ID NO: 22 - protein, 114 aa, Artificial Sequence
  Synthetic Sequence
EVQLLESGGGLVQPGGSLRLSCAAASGFTFSSYDMTWVRQAPGKGLEWVSTISGGGTYTYYQDSVKGRFTISRDNSKNTLYLQMNSLRAEDTAVYYCASMDYWGQGTTVTVSSA

SEQ ID NO: 23 - protein, 114 aa, Artificial Sequence
  Synthetic Sequence
EVQLLESGGGLVQPGGSLRLSCAADSGFTFSSYDMSWVRQAPGKGLEWVSTISGGGTYTYYQDSVKGRFTISRDNSKNTLYLQMNSLRAEDTAVYYCASMDYWGQGTTVTVSSA

SEQ ID NO: 24 - protein, 114 aa, Artificial Sequence
  Synthetic Sequence
EVQLLESGGGLVQPGGSLRLSCAAASGFTFSTYDMSWVRQAPGKGLEWVSTISGGGTYTYYQDSVKGRFTISRDNSKNTLYLQMNSLRAEDTAVYYCASMDYWGQGTTVTVSSA

SEQ ID NO: 25 - protein, 113 aa, Artificial Sequence
  Synthetic Sequence
EVQLLESGGGLVQPGGSLRLSCATSGFTFSSYDMSWVRQAPGKGLEWVSTISGGGTYTYYQDSVKGRFTISRDNSKNTLYLQMNSLRAEDTAVYYCASMDYWGQGTTVTVSSA

SEQ ID NO: 26 - protein, 113 aa, Artificial Sequence
  Synthetic Sequence
EVQLLESGGGLVQPGGSLRLSCAVSGFTFSSYDMSWVRQAPGKGLEWVSTISGGGTYTYYQDSVKGRFTISRDNSKNTLYLQMNSLRAEDTAVYYCASMDYWGQGTTVTVSSA

SEQ ID NO: 27 - protein, 114 aa, Artificial Sequence
  Synthetic Sequence
EVQLLESGGGLVQPGGSLRLSCAAGSGFTFSSYDMSWVRQAPGKGLEWVSTISGGGTYTYYQDSVKGRFTISRDNSKNTLYLQMNSLRAEDTAVYYCASMDYWGQGTTVTVSSA

SEQ ID NO: 28 - protein, 116 aa, Artificial Sequence
  Synthetic Sequence
EVQLLESGGGLVQPGGSLRLSCAASGFTFITFSSYDMSWVRQAPGKGLEWVSTISGGGTYTYYQDSVKGRFTISRDNSKNTLYLQMNSLRAEDTAVYYCASMDYWGQGTTVTVSSA

SEQ ID NO: 29 - protein, 113 aa, Artificial Sequence; identical to SEQ ID NO: 14
  Synthetic Sequence

SEQ ID NO: 30 - protein, 114 aa, Artificial Sequence
  Synthetic Sequence
EVQLLESGGGLVQPGGSLRLSCAAASGFTFSSYDMSWVRQAPGKGLEWVSTISGGGDYTYYQDSVKGRFTISRDNSKNTLYLQMNSLRAEDTAVYYCASMDYWGQGTTVTVSSA

SEQ ID NO: 31 - protein, 114 aa, Artificial Sequence
  Synthetic Sequence
EVQLLESGGGLVQPGGSLRLSCAAASGFTFSSYDMSWVRQAPGKGLEWVSTISGGGGYTYYQDSVKGRFTISRDNSKNTLYLQMNSLRAEDTAVYYCASMDYWGQGTTVTVSSA

SEQ ID NO: 32 - protein, 114 aa, Artificial Sequence
  Synthetic Sequence
EVQLLESGGGLVQPGGSLRLSCAAASGFTFSSYDMSWVRQAPGKGLEWVSTISGGGNYTYYQDSVKGRFTISRDNSKNTLYLQMNSLRAEDTAVYYCASMDYWGQGTTVTVSSA

SEQ ID NO: 33 - protein, 114 aa, Artificial Sequence
  Synthetic Sequence
EVQLLESGGGLVQPGGSLRLSCAAASGFTFSSYDMSWVRQAPGKGLEWVSTISGGGKYTYYQDSVKGRFTISRDNSKNTLYLQMNSLRAEDTAVYYCASMDYWGQGTTVTVSSA

SEQ ID NO: 34 - protein, 114 aa, Artificial Sequence
  Synthetic Sequence
EVQLLESGGGLVQPGGSLRLSCAAASGFTFSSYDMSWVRQAPGKGLDWVSTISGGGTYTYYQDSVKGRFTISRDNSKNTLYLQMNSLRAEDTAVYYCASMDYWGQGTTVTVSSA

SEQ ID NO: 35 - protein, 114 aa, Artificial Sequence
  Synthetic Sequence
EVQLLESGGGLVQPGGSLRLSCAAASGFTFSSYDMSWVRQAPGKGLDWVSTISGGGTYTYYQDSVKGRFTISRDNSKNTLYLQMNSLRAEDTAVYYCTSMDYWGQGTTVTVSSA

SEQ ID NO: 36 - protein, 114 aa, Artificial Sequence
  Synthetic Sequence
EVQLLESGGGLVQPGGSLRLSCAAASGFTFSSYDMSWVRQALGKGLEWVSTISGGGTYTYYQDSVKGRFTISRDNSKNTLYLQMNSLRAEDTAVYYCASMDYWGQGTTVTVSSA

SEQ ID NO: 37 - protein, 114 aa, Artificial Sequence
  Synthetic Sequence
EVQLLESGGGLVQPGGSLRLSCAAPSGFTFSSYDMSWVRQALGKGLEWVSTISGGGTYTYYQDSVKGRFTISRDNSKNTLYLQMNSLRAEDTAVYYCASMDYWGQGTTVTVSSA

SEQ ID NO: 38 - protein, 114 aa, Artificial Sequence
  Synthetic Sequence
EVQLLESGGGLVQPGGSLRLSCAAASGFTFSSYDMSWVRQALGKGLDWVSTISGGGTYTYYQDSVKGRFTISRDNSKNTLYLQMNSLRAEDTAVYYCASMDYWGQGTTVTVSSA

SEQ ID NO: 39 - protein, 114 aa, Artificial Sequence
  Synthetic Sequence
EVQLLESGGGLVQPGGSLRLSCAAPSGFTFSSYDMSWVRQALGKGLDWVSTISGGGTYTYYQDSVKGRFTISRDNSKNTLYLQMNSLRAEDTAVYYCASMDYWGQGTTVTVSSA

SEQ ID NO: 40 - protein, 113 aa, Artificial Sequence
  Synthetic Sequence
EVQLLESGGGLVQPGGSLRLSCAPSGFTFSSYDMSWVRQALGKGLEWVSTISGGGTYTYYQDSVKGRFTISRDNSKNTLYLQMNSLRAEDTAVYYCASMDYWGQGTTVTVSSA

SEQ ID NO: 41 - protein, 113 aa, Artificial Sequence
  Synthetic Sequence
EVQLLESGGGLVQPGGSLRLSCAPSGFTFSSYDMSWVRQALGKGLDWVSTISGGGTYTYYQDSVKGRFTISRDNSKNTLYLQMNSLRAEDTAVYYCASMDYWGQGTTVTVSSA

SEQ ID NO: 42 - protein, 113 aa, Artificial Sequence
  Synthetic Sequence
EVQLLESGGGLVQPGGSLRLSCAPSGFTFSSYDMSWVRQAPGKGLDWVSTISGGGTYTYYQDSVKGRFTISRDNSKNTLYLQMNSLRAEDTAVYYCASMDYWGQGTTVTVSSA

SEQ ID NO: 43 - protein, 114 aa, Artificial Sequence
  Synthetic Sequence
EVQLLESGGGLVQPGGSLRLSCAAASGFTFSSYDMSWVRQAPGKGLDWVSTISGGGTYTYYQDSVKGRFTISRDNSKNTLYLQMNSLRVEDTAVYYCASMDYWGQGTTVTVSSA

SEQ ID NO: 44 - protein, 114 aa, Artificial Sequence
  Synthetic Sequence
EVQLLESGGGLVQPGGSLRLSCAAASGFTFSSYDMSWVRQALGKGLDWVSTISGGGTYTYYQDSVKGRFTISRDNSKNTLYLQMNSLRVEDTAVYYCASMDYWGQGTTVTVSSA

SEQ ID NO: 45 - protein, 108 aa, Artificial Sequence
  Synthetic Sequence
  MISC_FEATURE (6)..(6): Xaa1 is glutamine (Gln) or histidine (His)
  MISC_FEATURE (25)..(25): Xaa2 is alanine (Ala) or threonine (Thr)
  MISC_FEATURE (30)..(30): Xaa3 is serine (Ser), arginine (Arg), asparagine (Asn), or threonine (Thr)
  MISC_FEATURE (31)..(31): Xaa4 is serine (Ser), arginine (Arg), aspartic acid (Asp), threonine (Thr), or glycine (Gly)
  MISC_FEATURE (37)..(37): Xaa5 is glutamine (Gln) or histidine (His)
  MISC_FEATURE (40)..(40): Xaa6 is proline (Pro) or alanine (Ala)
  MISC_FEATURE (41)..(41): Xaa7 is glycine (Gly), lysine (Lys), or arginine (Arg)
  MISC_FEATURE (48)..(48): Xaa8 is isoleucine (Ile) or methionine (Met)
  MISC_FEATURE (50)..(50): Xaa9 is alanine (Ala), glycine (Gly), aspartic acid (Asp), threonine (Thr), serine (Ser), valine (Val), or isoleucine (Ile)
  MISC_FEATURE (53)..(53): Xaa10 is serine (Ser) or threonine (Thr)
  MISC_FEATURE (85)..(85): Xaa11 is valine (Val), methionine (Met), or alanine (Ala)
  MISC_FEATURE (91)..(91): Xaa12 is serine (ser) or arginine (Arg)
  MISC_FEATURE (92)..(92): Xaa13 is tyrosine (Tyr), histidine (His), phenylalanine (Phe), aspartic acid (Asp), serine (Ser), or asparagine (Asn)
  MISC_FEATURE (93)..(93): Xaa14 is serine (Ser) or asparagine (Asn)
  MISC_FEATURE (94)..(94): Xaa15 is threonine (Thr), serine (Ser), alanine (Ala), or proline (Pro)
  MISC_FEATURE (96)..(96): Xaa16 is leucine (Leu) or histidine (His)
  MISC_FEATURE (100)..(100): Xaa17 is glycine (Gly), arginine (Arg), or glutamic acid (Glu)
  MISC_FEATURE (104)..(104): Xaa18 is valine (Val) or leucine (Leu)
DIQMTXSPSSLSASVGDRVTITCRXSQSIXXYLNWYXQKXXKAPKLLXYXASXLQSGVPSRFSGSGSGTDFTLTISSLQPEDFAXYYCQQXXXXPXTFGXGTKXEIKR

SEQ ID NO: 46 - protein, 108 aa, Artificial Sequence
  Synthetic Sequence
DIQMTQSPSSLSASVGDRVTITCRASQSISSYLNWYQQKPGKAPKLLIYAASSLQSGVPSRFSGSGSGTDFTLTISSLQPEDFAVYYCQQSYSTPLTFGGGTKVEIKR

SEQ ID NO: 47 - protein, 108 aa, Artificial Sequence
  Synthetic Sequence
DIQMTQSPSSLSASVGDRVTITCRASQSISSYLNWYQQKPGKAPKLLIYAASSLQSGVPSRFSGSGSGTDFTLTISSLQPEDFAVYYCQQSYSSPLTFGGGTKVEIKR

SEQ ID NO: 48 - protein, 108 aa, Artificial Sequence
  Synthetic Sequence
DIQMTQSPSSLSASVGDRVTITCRASQSISRYLNWYQQKPGKAPKLLIYAASSLQSGVPSRFSGSGSGTDFTLTISSLQPEDFAVYYCQQSYSSPLTFGGGTKVEIKR

SEQ ID NO: 49 - protein, 108 aa, Artificial Sequence
  Synthetic Sequence
DIQMTQSPSSLSASVGDRVTITCRASQSISRYLNWYQQKPGKAPKLLIYGASSLQSGVPSRFSGSGSGTDFTLTISSLQPEDFAVYYCQQSYSSPLTFGGGTKVEIKR

SEQ ID NO: 50 - protein, 108 aa, Artificial Sequence
  Synthetic Sequence
DIQMTQSPSSLSASVGDRVTITCRASQSIRRYLNWYQQKPGKAPKLLIYAASSLQSGVPSRFSGSGSGTDFTLTISSLQPEDFAVYYCQQSYSSPLTFGGGTKVEIKR

SEQ ID NO: 51 - protein, 108 aa, Artificial Sequence
  Synthetic Sequence
DIQMTQSPSSLSASVGDRVTITCRASQSIRRYLNWYQQKPGKAPKLLIYGASSLQSGVPSRFSGSGSGTDFTLTISSLQPEDFAVYYCQQSYSSPLTFGGGTKVEIKR

SEQ ID NO: 52 - protein, 108 aa, Artificial Sequence
  Synthetic Sequence
DIQMTQSPSSLSASVGDRVTITCRASQSINRYLNWYQQKPGKAPKLLIYAASSLQSGVPSRFSGSGSGTDFTLTISSLQPEDFAVYYCQQSYSSPLTFGGGTKVEIKR

SEQ ID NO: 53 - protein, 108 aa, Artificial Sequence
  Synthetic Sequence
DIQMTQSPSSLSASVGDRVTITCRASQSISRYLNWYQQKPGKAPKLLIYAASSLQSGVPSRFSGSGSGTDFTLTISSLQPEDFAVYYCQQSHSSPLTFGGGTKVEIKR

SEQ ID NO: 54 - protein, 108 aa, Artificial Sequence
  Synthetic Sequence
DIQMTQSPSSLSASVGDRVTITCRASQSINRYLNWYQQKPGKAPKLLIYGASSLQSGVPSRFSGSGSGTDFTLTISSLQPEDFAVYYCQQSYSSPLTFGGGTKVEIKR

SEQ ID NO: 55 - protein, 108 aa, Artificial Sequence
  Synthetic Sequence
DIQMTQSPSSLSASVGDRVTITCRASQSIRRYLNWYQQKPGKAPKLLIYGASSLQSGVPSRFSGSGSGTDFTLTISSLQPEDFAVYYCQQSHSSPLTFGGGTKVEIKR

SEQ ID NO: 56 - protein, 108 aa, Artificial Sequence
  Synthetic Sequence
DIQMTQSPSSLSASVGDRVTITCRASQSIRRYLNWYQQKPGKAPKLLIYGASSLQSGVPSRFSGSGSGTDFTLTISSLQPEDFAVYYCQQSYSSPHTFGGGTKVEIKR

SEQ ID NO: 57 - protein, 108 aa, Artificial Sequence
  Synthetic Sequence
DIQMTQSPSSLSASVGDRVTITCRASQSIRRYLNWYQQKPGKAPKLLIYGASSLQSGVPSRFSGSGSGTDFTLTISSLQPEDFAVYYCQQSYSAPLTFGGGTKVEIKR

SEQ ID NO: 58 - protein, 108 aa, Artificial Sequence
  Synthetic Sequence
DIQMTQSPSSLSASVGDRVTITCRASQSIRRYLNWYQQKPGKAPKLLIYAASSLQSGVPSRFSGSGSGTDFTLTISSLQPEDFAVYYCQQSYSAPLTFGGGTKVEIKR

SEQ ID NO: 59 - protein, 108 aa, Artificial Sequence
  Synthetic Sequence
DIQMTQSPSSLSASVGDRVTITCRASQSISRYLNWYQQKPGKAPKLLIYAASSLQSGVPSRFSGSGSGTDFTLTISSLQPEDFAVYYCQQSHSAPLTFGGGTKVEIKR

SEQ ID NO: 60 - protein, 108 aa, Artificial Sequence
  Synthetic Sequence
DIQMTQSPSSLSASVGDRVTITCRASQSINRYLNWYQQKPGKAPKLLIYGASSLQSGVPSRFSGSGSGTDFTLTISSLQPEDFAVYYCQQSYSAPLTFGGGTKVEIKR

SEQ ID NO: 61 - protein, 108 aa, Artificial Sequence
  Synthetic Sequence
DIQMTQSPSSLSASVGDRVTITCRASQSIRRYLNWYQQKPGKAPKLLIYGASSLQSGVPSRFSGSGSGTDFTLTISSLQPEDFAVYYCQQSHSAPLTFGGGTKVEIKR

SEQ ID NO: 62 - protein, 108 aa, Artificial Sequence
  Synthetic Sequence
DIQMTQSPSSLSASVGDRVTITCRASQSIRRYLNWYQQKPGKAPKLLIYGASSLQSGVPSRFSGSGSGTDFTLTISSLQPEDFAVYYCQQSYSSPLTFGRGTKVEIKR

SEQ ID NO: 63 - protein, 108 aa, Artificial Sequence
  Synthetic Sequence
DIQMTQSPSSLSASVGDRVTITCRASQSIRRYLNWYQQKPGKAPKLLIYGASSLQSGVPSRFSGSGSGTDFTLTISSLQPEDFAMYYCQQSYSSPLTFGGGTKVEIKR

SEQ ID NO: 64 - protein, 108 aa, Artificial Sequence
  Synthetic Sequence
DIQMTQSPSSLSASVGDRVTITCRASQSIRRYLNWYQQKPGKAPKLLIYGASSLQSGVPSRFSGSGSGTDFTLTISSLQPEDFAVYYCQQSHSNPLTFGGGTKVEIKR

SEQ ID NO: 65 - protein, 108 aa, Artificial Sequence
  Synthetic Sequence
DIQMTQSPSSLSASVGDRVTITCRASQSIRRYLNWYQQKPGKAPKLLIYGASSLQSGVPSRFSGSGSGTDFTLTISSLQPEDFAVYYCQQSHSMPLTFGGGTKVEIKR

SEQ ID NO: 66 - protein, 108 aa, Artificial Sequence
  Synthetic Sequence
DIQMTQSPSSLSASVGDRVTITCRASQSIRRYLNWYQQKPGKAPKLLIYGASSLQSGVPSRFSGSGSGTDFTLTISSLQPEDFAVYYCQQSHSIPLTFGGGTKVEIKR

SEQ ID NO: 67 - protein, 108 aa, Artificial Sequence
  Synthetic Sequence
DIQMTQSPSSLSASVGDRVTITCRASQSIRRYLNWYQQKPGKAPKLLIYGASSLQSGVPSRFSGSGSGTDFTLTISSLQPEDFAVYYCQQSHSLPLTFGGGTKVEIKR

SEQ ID NO: 68 - protein, 108 aa, Artificial Sequence
  Synthetic Sequence
DIQMTQSPSSLSASVGDRVTITCRASQSIRRYLNWYQQKPGKAPKLLIYGASSLQSGVPSRFSGSGSGTDFTLTISSLQPEDFAVYYCQQSHSRPLTFGGGTKVEIKR

SEQ ID NO: 69 - protein, 108 aa, Artificial Sequence
  Synthetic Sequence
DIQMTQSPSSLSASVGDRVTITCRASQSIRRYLNWYQQKPGKAPKLLIYGASSLQSGVPSRFSGSGSGTDFTLTISSLQPEDFAVYYCQQSYSSPLTFGEGTKVEIKR

SEQ ID NO: 70 - protein, 108 aa, Artificial Sequence
  Synthetic Sequence
DIQMTQSPSSLSASVGDRVTITCRASQSIRRYLNWYQQKPGKAPKLLIYGASSLQSGVPSRFSGSGSGTDFTLTISSLQPEDFAVYYCQQSYSSPLTFGGGTKLEIKR

SEQ ID NO: 71 - protein, 108 aa, Artificial Sequence
  Synthetic Sequence
DIQMTQSPSSLSASVGDRVTITCRASQSIRRYLNWYQQKPGKAPKLLIYGASSLQSGVPSRFSGSGSGTDFTLTISSLQPEDFAAYYCQQSYSSPLTFGGGTKVEIKR

SEQ ID NO: 72 - protein, 108 aa, Artificial Sequence
  Synthetic Sequence
DIQMTQSPSSLSASVGDRVTITCRASQSIRRYLNWYQQKPKKAPKLLIYGASSLQSGVPSRFSGSGSGTDFTLTISSLQPEDFAVYYCQQSHSSPLTFGGGTKVEIKR

SEQ ID NO: 73 - protein, 108 aa, Artificial Sequence
  Synthetic Sequence
DIQMTQSPSSLSASVGDRVTITCRASQSIRRYLNWYQQKPRKAPKLLIYGASSLQSGVPSRFSGSGSGTDFTLTISSLQPEDFAVYYCQQSHSSPLTFGGGTKVEIKR

SEQ ID NO: 74 - protein, 108 aa, Artificial Sequence; identical to SEQ ID NO: 55
  Synthetic Sequence

SEQ ID NO: 75 - protein, 108 aa, Artificial Sequence
  Synthetic Sequence
DIQMTQSPSSLSASVGDRVTITCRASQSIRRYLNWYQQKPGKAPKLLIYGASSLQSGVPSRFSGSGSGTDFTLTISSLQPEDFAVYYCQQSHSPPLTFGGGTKVEIKR

SEQ ID NO: 76 - protein, 108 aa, Artificial Sequence
  Synthetic Sequence
DIQMTQSPSSLSASVGDRVTITCRASQSITRYLNWYQQKPGKAPKLLIYGASSLQSGVPSRFSGSGSGTDFTLTISSLQPEDFAVYYCQQSHSSPLTFGGGTKVEIKR

SEQ ID NO: 77 - protein, 108 aa, Artificial Sequence
  Synthetic Sequence
DIQMTQSPSSLSASVGDRVTITCRASQSINRYLNWYQQKPGKAPKLLIYGASSLQSGVPSRFSGSGSGTDFTLTISSLQPEDFAVYYCQQSHSSPLTFGGGTKVEIKR

SEQ ID NO: 78 - protein, 108 aa, Artificial Sequence
  Synthetic Sequence
DIQMTQSPSSLSASVGDRVTITCRASQSIRDYLNWYQQKPGKAPKLLIYGASSLQSGVPSRFSGSGSGTDFTLTISSLQPEDFAVYYCQQSHSSPLTFGGGTKVEIKR

SEQ ID NO: 79 - protein, 108 aa, Artificial Sequence
  Synthetic Sequence
DIQMTQSPSSLSASVGDRVTITCRASQSIRTYLNWYQQKPGKAPKLLIYGASSLQSGVPSRFSGSGSGTDFTLTISSLQPEDFAVYYCQQSHSSPLTFGGGTKVEIKR

SEQ ID NO: 80 - protein, 108 aa, Artificial Sequence
  Synthetic Sequence
DIQMTQSPSSLSASVGDRVTITCRASQSIRGYLNWYQQKPGKAPKLLIYGASSLQSGVPSRFSGSGSGTDFTLTISSLQPEDFAVYYCQQSHSSPLTFGGGTKVEIKR

SEQ ID NO: 81 - protein, 108 aa, Artificial Sequence
  Synthetic Sequence
DIQMTQSPSSLSASVGDRVTITCRASQSIRRYLNWYQQKPGKAPKLLIYDASSLQSGVPSRFSGSGSGTDFTLTISSLQPEDFAVYYCQQSHSSPLTFGGGTKVEIKR

SEQ ID NO: 82 - protein, 108 aa, Artificial Sequence
  Synthetic Sequence
DIQMTQSPSSLSASVGDRVTITCRASQSIRRYLNWYQQKPGKAPKLLIYTASSLQSGVPSRFSGSGSGTDFTLTISSLQPEDFAVYYCQQSHSSPLTFGGGTKVEIKR

SEQ ID NO: 83 - protein, 108 aa, Artificial Sequence
  Synthetic Sequence
DIQMTQSPSSLSASVGDRVTITCRASQSIRRYLNWYQQKPGKAPKLLIYSASSLQSGVPSRFSGSGSGTDFTLTISSLQPEDFAVYYCQQSHSSPLTFGGGTKVEIKR

SEQ ID NO: 84 - protein, 108 aa, Artificial Sequence
  Synthetic Sequence
DIQMTQSPSSLSASVGDRVTITCRASQSIRRYLNWYQQKPGKAPKLLIYVASSLQSGVPSRFSGSGSGTDFTLTISSLQPEDFAVYYCQQSHSSPLTFGGGTKVEIKR

SEQ ID NO: 85 - protein, 108 aa, Artificial Sequence
  Synthetic Sequence
DIQMTQSPSSLSASVGDRVTITCRASQSIRRYLNWYQQKPGKAPKLLIYIASSLQSGVPSRFSGSGSGTDFTLTISSLQPEDFAVYYCQQSHSSPLTFGGGTKVEIKR

SEQ ID NO: 86 - protein, 108 aa, Artificial Sequence
  Synthetic Sequence
DIQMTQSPSSLSASVGDRVTITCRASQSIRRYLNWYQQKPGKAPKLLIYGASSLQSGVPSRFSGSGSGTDFTLTISSLQPEDFAVYYCQQSFSSPLTFGGGTKVEIKR

SEQ ID NO: 87 - protein, 108 aa, Artificial Sequence
  Synthetic Sequence
DIQMTQSPSSLSASVGDRVTITCRASQSIRRYLNWYQQKPGKAPKLLIYGASSLQSGVPSRFSGSGSGTDFTLTISSLQPEDFAVYYCQQSDSSPLTFGGGTKVEIKR

SEQ ID NO: 88 - protein, 108 aa, Artificial Sequence
  Synthetic Sequence
DIQMTQSPSSLSASVGDRVTITCRASQSIRRYLNWYQQKPGKAPKLLIYGASSLQSGVPSRFSGSGSGTDFTLTISSLQPEDFAVYYCQQSSSSPLTFGGGTKVEIKR

SEQ ID NO: 89 - protein, 108 aa, Artificial Sequence
  Synthetic Sequence
DIQMTQSPSSLSASVGDRVTITCRASQSIRRYLNWYQQKPGKAPKLLIYGASSLQSGVPSRFSGSGSGTDFTLTISSLQPEDFAVYYCQQSNSSPLTFGGGTKVEIKR

SEQ ID NO: 90 - protein, 108 aa, Artificial Sequence
  Synthetic Sequence
DIQMTQSPSSLSASVGDRVTITCRASQSIRRYLNWYHQKPGKAPKLLIYGASSLQSGVPSRFSGSGSGTDFTLTISSLQPEDFAVYYCQQSHSSPLTFGGGTKVEIKR

SEQ ID NO: 91 - protein, 108 aa, Artificial Sequence
  Synthetic Sequence
DIQMTQSPSSLSASVGDRVTITCRASQSIRRYLNWYHQKPGKAPKLLIYGASSLQSGVPSRFSGSGSGTDFTLTISSLQPEDFAVYYCQQSHSAPLTFGGGTKVEIKR

SEQ ID NO: 92 - protein, 108 aa, Artificial Sequence
  Synthetic Sequence
DIQMTQSPSSLSASVGDRVTITCRASQSIRRYLNWYHQKPKKAPKLLIYGASSLQSGVPSRFSGSGSGTDFTLTISSLQPEDFAVYYCQQSHSSPLTFGGGTKVEIKR

SEQ ID NO: 93 - protein, 108 aa, Artificial Sequence
  Synthetic Sequence
DIQMTQSPSSLSASVGDRVTITCRTSQSIRRYLNWYQQKPGKAPKLLIYGASSLQSGVPSRFSGSGSGTDFTLTISSLQPEDFAVYYCQQSHSSPLTFGGGTKVEIKR

SEQ ID NO: 94 - protein, 108 aa, Artificial Sequence
  Synthetic Sequence
DIQMTHSPSSLSASVGDRVTITCRASQSIRRYLNWYQQKPGKAPKLLIYGASSLQSGVPSRFSGSGSGTDFTLTISSLQPEDFAVYYCQQSHSSPLTFGGGTKVEIKR

SEQ ID NO: 95 - protein, 108 aa, Artificial Sequence
  Synthetic Sequence
DIQMTHSPSSLSASVGDRVTITCRASQSIRRYLNWYQQKPKKAPKLLIYGASSLQSGVPSRFSGSGSGTDFTLTISSLQPEDFAVYYCQQSHSSPLTFGGGTKVEIKR

SEQ ID NO: 96 - protein, 108 aa, Artificial Sequence
  Synthetic Sequence
DIQMTQSPSSLSASVGDRVTITCRASQSIRRYLNWYQQKPGKAPKLLIYGASSLQSGVPSRFSGSGSGTDFTLTISSLQPEDFAVYYCQQSHNSPLTFGGGTKVEIKR

SEQ ID NO: 97 - protein, 108 aa, Artificial Sequence
  Synthetic Sequence
DIQMTQSPSSLSASVGDRVTITCRASQSIRRYLNWYQQKPGKAPKLLMYGASSLQSGVPSRFSGSGSGTDFTLTISSLQPEDFAVYYCQQSHSSPLTFGGGTKVEIKR

SEQ ID NO: 98 - protein, 108 aa, Artificial Sequence
  Synthetic Sequence
DIQMTQSPSSLSASVGDRVTITCRASQSIRRYLNWYQQKPGKAPKLLMYGASSLQSGVPSRFSGSGSGTDFTLTISSLQPEDFAVYYCQQSHSAPLTFGGGTKVEIKR

SEQ ID NO: 99 - protein, 108 aa, Artificial Sequence
  Synthetic Sequence
DIQMTQSPSSLSASVGDRVTITCRASQSISRYLNWYQQKPGKAPKLLMYAASSLQSGVPSRFSGSGSGTDFTLTISSLQPEDFAVYYCQQSYSSPLTFGGGTKVEIKR

SEQ ID NO: 100 - protein, 108 aa, Artificial Sequence
  Synthetic Sequence
DIQMTQSPSSLSASVGDRVTITCRTSQSIRRYLNWYQQKPKKAPKLLIYGASSLQSGVPSRFSGSGSGTDFTLTISSLQPEDFAVYYCQQSHSSPLTFGGGTKVEIKR

SEQ ID NO: 101 - protein, 108 aa, Artificial Sequence
  Synthetic Sequence
DIQMTQSPSSLSASVGDRVTITCRASQSIRRYLNWYHQKPGKAPKLLIYGASSLQSGVPSRFSGSGSGTDFTLTISSLQPEDFAVYYCQQSHNAPLTFGGGTKVEIKR

SEQ ID NO: 102 - protein, 108 aa, Artificial Sequence
  Synthetic Sequence
DIQMTQSPSSLSASVGDRVTITCRTSQSIRRYLNWYHQKPGKAPKLLIYGASSLQSGVPSRFSGSGSGTDFTLTISSLQPEDFAVYYCQQSHSAPLTFGGGTKVEIKR

SEQ ID NO: 103 - protein, 108 aa, Artificial Sequence
  Synthetic Sequence
DIQMTQSPSSLSASVGDRVTITCRASQSIRRYLNWYHQKPGKAPKLLMYGASSLQSGVPSRFSGSGSGTDFTLTISSLQPEDFAVYYCQQSHSAPLTFGGGTKVEIKR

SEQ ID NO: 104 - protein, 108 aa, Artificial Sequence
  Synthetic Sequence
DIQMTQSPSSLSASVGDRVTITCRASQSIRRYLNWYHQKAGKAPKLLIYGASSLQSGVPSRFSGSGSGTDFTLTISSLQPEDFAVYYCQQSHSAPLTFGGGTKVEIKR

SEQ ID NO: 105 - protein, 108 aa, Artificial Sequence
  Synthetic Sequence
DIQMTHSPSSLSASVGDRVTITCRASQSIRRYLNWYHQKPGKAPKLLIYGASSLQSGVPSRFSGSGSGTDFTLTISSLQPEDFAVYYCQQSHSAPLTFGGGTKVEIKR

SEQ ID NO: 106 - protein, 108 aa, Artificial Sequence
  Synthetic Sequence
DIQMTHSPSSLSASVGDRVTITCRASQSIRRYLNWYHQKAGKAPKLLIYGASSLQSGVPSRFSGSGSGTDFTLTISSLQPEDFAVYYCQQSHSAPLTFGGGTKVEIKR

SEQ ID NO: 107 - protein, 108 aa, Artificial Sequence
  Synthetic Sequence
DIQMTHSPSSLSASVGDRVTITCRASESIRRYLNWYHQKPGKAPKLLIYGASSLQSGVPSRFSGSGSGTDFTLTISSLQPEDFAVYYCQQSHSAPLTFGGGTKVEIKR

SEQ ID NO: 108 - protein, 108 aa, Artificial Sequence
  Synthetic Sequence
DIQMTHSPSSLSASVGDRVTITCRASESIRRYLNWYHQKAGKAPKLLIYGASSLQSGVPSRFSGSGSGTDFTLTISSLQPEDFAVYYCQQSHSAPLTFGGGTKVEIKR

SEQ ID NO: 109 - protein, 108 aa, Artificial Sequence
  Synthetic Sequence
DIQMTHSPSSLSASVGDRVTITCRASQSIRRYLNWYHQKPGKAPKLLMYGASSLQSGVPSRFSGSGSGTDFTLTISSLQPEDFAVYYCQQSHNAPLTFGGGTKVEIKR

SEQ ID NO: 110 - protein, 108 aa, Artificial Sequence
  Synthetic Sequence
DIQMTHSPSSLSASVGDRVTITCRASQSIRRYLNWYHQKPGKAPKLLMYGASSLQSGVPSRFSGSGSGTDFTLTISSLQPEDFAVYYCQQSHSAPLTFGGGTKVEIKR

SEQ ID NO: 111 - protein, 108 aa, Artificial Sequence
  Synthetic Sequence
DIQMTHSPSSLSASVGDRVTITCRASQSIRRYLNWYHQKAGKAPKLLMYGASSLQSGVPSRFSGSGSGTDFTLTISSLQPEDFAVYYCQQSHNAPLTFGGGTKVEIKR

SEQ ID NO: 112 - protein, 108 aa, Artificial Sequence
  Synthetic Sequence
DIQMTQSPSSLSASVGDRVTITCRASQSIRRYLNWYHQKPGKAPKLLMYGASSLQSGVPSRFSGSGSGTDFTLTISSLQPEDFAVYYCQQRHSAPLTFGGGTKVEIKR

SEQ ID NO: 113 - protein, 108 aa, Artificial Sequence
  Synthetic Sequence
DIQMTQSPSSLSASVGDRVTITCRASQSIRRYLNWYHQKPGKAPKLLIYGASSLQSGVPSRFSGSGSGTDFTLTISSLQPEDFAVYYCQQRHNAPLTFGGGTKVEIKR

SEQ ID NO: 114 - protein, 108 aa, Artificial Sequence
  Synthetic Sequence
DIQMTHSPSSLSASVGDRVTITCRASQSIRRYLNWYHQKPGKAPKLLIYGASSLQSGVPSRFSGSGSGTDFTLTISSLQPEDFAVYYCQQRHSAPLTFGGGTKVEIKR

SEQ ID NO: 115 - protein, 108 aa, Artificial Sequence
  Synthetic Sequence
DIQMTQSPSSLSASVGDRVTITCRASQSIRRYLNWYHQKPGKAPKLLIYGASTLQSGVPSRFSGSGSGTDFTLTISSLQPEDFAVYYCQQSHSAPLTFGGGTKVEIKR

SEQ ID NO: 116 - protein, 108 aa, Artificial Sequence
  Synthetic Sequence
DIQMTQSPSSLSASVGDRVTITCRASQSIRRYLNWYHQKPGKAPKLLMYGASTLQSGVPSRFSGSGSGTDFTLTISSLQPEDFAVYYCQQRHSAPLTFGGGTKVEIKR

SEQ ID NO: 117 - protein, 108 aa, Artificial Sequence
  Synthetic Sequence
DIQMTHSPSSLSASVGDRVTITCRASQSIRRYLNWYHQKPGKAPKLLMYGASTLQSGVPSRFSGSGSGTDFTLTISSLQPEDFAVYYCQQRHSAPLTFGGGTKVEIKR

SEQ ID NO: 118 - protein, 108 aa, Artificial Sequence
  Synthetic Sequence
DIQMTQSPSSLSASVGDRVTITCRASQSIRRYLNWYHQKPGKAPKLLIYGASTLQSGVPSRFSGSGSGTDFTLTISSLQPEDFAVYYCQQRHNAPLTFGGGTKVEIKR

SEQ ID NO: 119 - protein, 108 aa, Artificial Sequence
  Synthetic Sequence
DIQMTHSPSSLSASVGDRVTITCRASQSIRRYLNWYHQKPGKAPKLLIYGASTLQSGVPSRFSGSGSGTDFTLTISSLQPEDFAVYYCQQRHNAPLTFGGGTKVEIKR

SEQ ID NO: 120 - protein, 108 aa, Artificial Sequence
  Synthetic Sequence
DIQMTHSPSSLSASVGDRVTITCRASQSIRRYLNWYHQKPGKAPKLLMYGASTLQSGVPSRFSGSGSGTDFTLTISSLQPEDFAVYYCQQSHNAPLTFGGGTKVEIKR

SEQ ID NO: 121 - protein, 108 aa, Artificial Sequence
  Synthetic Sequence
DIQMTQSPSSLSASVGDRVTITCRASQSIRRYLNWYHQKPGKAPKLLMYGASSLQSGVPSRFSGSGSGTDFTLTISSLQPEDFAVYYCQQSHNAPLTFGGGTKVEIKR

SEQ ID NO: 122 - protein, 108 aa, Artificial Sequence
  Synthetic Sequence
DIQMTHSPSSLSASVGDRVTITCRASQSIRRYLNWYHQKPGKAPKLLIYGASSLQSGVPSRFSGSGSGTDFTLTISSLQPEDFAVYYCQQSHNAPLTFGGGTKVEIKR

SEQ ID NO: 123 - protein, 108 aa, Artificial Sequence
  Synthetic Sequence
DIQMTQSPSSLSASVGDRVTITCRASQSIRRYLNWYHQKPGKAPKLLMYGASTLQSGVPSRFSGSGSGTDFTLTISSLQPEDFAVYYCQQSHSAPLTFGGGTKVEIKR

SEQ ID NO: 124 - protein, 108 aa, Artificial Sequence
  Synthetic Sequence
DIQMTQSPSSLSASVGDRVTITCRASQSIRRYLNWYHQKPGKAPKLLIYGASTLQSGVPSRFSGSGSGTDFTLTISSLQPEDFAVYYCQQSHNAPLTFGGGTKVEIKR

SEQ ID NO: 125 - protein, 108 aa, Artificial Sequence
  Synthetic Sequence
DIQMTHSPSSLSASVGDRVTITCRASQSIRRYLNWYHQKPGKAPKLLIYGASTLQSGVPSRFSGSGSGTDFTLTISSLQPEDFAVYYCQQSHSAPLTFGGGTKVEIKR

SEQ ID NO: 126 - protein, 123 aa, Artificial Sequence
  Synthetic Sequence
  MISC_FEATURE (4)..(4): Xaa1 is leucine (Leu), valine (Val), or methionine (Met)
  MISC_FEATURE (6)..(8): the subsequence Xaa2 Xaa3 Xaa4 is deleted or is Glu-Ser-Leu
  MISC_FEATURE (9)..(9): Xaa5 is deleted or is glutamic acid (Glu)
  MISC_FEATURE (13)..(13): Xaa6 is glycine (Gly) or aspartic acid (Asp)
  MISC_FEATURE (15)..(15): Xaa7 is valine (Val) or isoleucine (Ile)
  MISC_FEATURE (24)..(24): Xaa8 is serine (Ser) or tyrosine (Tyr)
  MISC_FEATURE (26)..(26): Xaa9 is alanine (Ala) or valine (Val)
  MISC_FEATURE (33)..(33): Xaa10 is serine (Ser), asparagine (Asn), arginine (Arg), threonine (Thr), aspartic acid (Asp), or glycine (Gly)
  MISC_FEATURE (34)..(34): Xaa11 is deleted or is glycine (Gly)
  MISC_FEATURE (37)..(37): Xaa12 is alanine (Ala) or threonine (Thr)
  MISC_FEATURE (39)..(39): Xaa13 is serine (Ser) or asparagine (Asn)
  MISC_FEATURE (54)..(54): Xaa14 is alanine (Ala), glycine (Gly), valine (Val), serine (Ser), phenylalanine (Phe), isoleucine (Ile), threonine (Thr), or aspartic acid (Asp)
  MISC_FEATURE (61)..(61): Xaa15 is serine (Ser) or asparagine (Asn)
  MISC_FEATURE (65)..(65): Xaa16 is alanine (Ala), valine (Val), or asparagine (Asn)
  MISC_FEATURE (71)..(71): Xaa17 is arginine (Arg) or glutamine (Gln)
  MISC_FEATURE (76)..(76): Xaa18 is arginine (Arg) or lysine (Lys)
  MISC_FEATURE (80)..(80): Xaa19 is lysine (Lys) or asparagine (Asn)
  MISC_FEATURE (83)..(83): Xaa20 is leucine (Leu), valine (Val), threonine (Thr), methionine (Met), or proline (Pro)
  MISC_FEATURE (89)..(89): Xaa21 is serine (Ser) or asparagine (Asn)
  MISC_FEATURE (101)..(101): Xaa22 is alanine (Ala) or glycine (Gly)
  MISC_FEATURE (106)..(106): Xaa23 is glycine (Gly), valine (Val), aspartic acid (Asp), alanine (Ala), threonine (Thr), or asparagine (Asn)
  MISC_FEATURE (107)..(107): Xaa24 is glycine (Gly), serine (Ser), valine (Val), aspartic acid (Asp), asparagine (Asn), or threonine (Thr)
  MISC_FEATURE (113)..(113): Xaa25 is glycine (Gly) or aspartic acid (Asp)
EVQXLXXXXSGGXLXQPGGSLRLXCXASGFTFXXSYXMXWVRQAPGKGLEWVSXISGSGGXTYYXDSVKGXFTISXDNSXNTXYLQMNXLRAEDTAVYYCXKKYYXXPADYWXQGTLVTVSSG

SEQ ID NO: 127 - protein, 119 aa, Artificial Sequence
  Synthetic Sequence
EVQLLESGGGLVQPGGSLRLSCAASGFTFSSYAMSWVRQAPGKGLEWVSAISGSGGSTYYADSVKGRFTISRDNSKNTLYLQMNSLRAEDTAVYYCAKKYYGGPADYWGQGTLVTVSSG

SEQ ID NO: 128 - protein, 119 aa, Artificial Sequence
  Synthetic Sequence
EVQLLESGGGLVQPGGSLRLSCAASGFTFSSYAMSWVRQAPGKGLEWVSAISGSGGSTYYADSVKGRFTISRDNSKNTLYLQMNSLRAEDTAVYYCAKKYYVGPADYWGQGTLVTVSSG

SEQ ID NO: 129 - protein, 119 aa, Artificial Sequence
  Synthetic Sequence
EVQLLESGGGLVQPGGSLRLSCAASGFTFNSYAMSWVRQAPGKGLEWVSAISGSGGSTYYADSVKGRFTISRDNSKNTLYLQMNSLRAEDTAVYYCAKKYYVGPADYWGQGTLVTVSSG

SEQ ID NO: 130 - protein, 119 aa, Artificial Sequence
  Synthetic Sequence
EVQLLESGGGLVQPGGSLRLSCAASGFTFSSYAMSWVRQAPGKGLEWVSAISGSGGSTYYADSVKGRFTISRDNSNNTLYLQMNSLRAEDTAVYYCAKKYYVGPADYWGQGTLVTVSSG

SEQ ID NO: 131 - protein, 119 aa, Artificial Sequence
  Synthetic Sequence
EVQLLESGGGLVQPGGSLRLSCAASGFTFSSYAMSWVRQAPGKGLEWVSGISGSGGSTYYADSVKGRFTISRDNSKNTLYLQMNSLRAEDTAVYYCAKKYYVGPADYWGQGTLVTVSSG

SEQ ID NO: 132 - protein, 119 aa, Artificial Sequence
  Synthetic Sequence
EVQLLESGGGLVQPGGSLRLSCAASGFTFNSYAMSWVRQAPGKGLEWVSAISGSGGSTYYADSVKGRFTISRDNSKNTLYLQMNSLRAEDTAVYYCAKKYYDGPADYWGQGTLVTVSSG

SEQ ID NO: 133 - protein, 119 aa, Artificial Sequence
  Synthetic Sequence
EVQLLESGGGLVQPGGSLRLSCAASGFTFNSYAMSWVRQAPGKGLEWVSAISGSGGSTYYADSVKGRFTISKDNSKNTLYLQMNSLRAEDTAVYYCAKKYYVGPADYWGQGTLVTVSSG

SEQ ID NO: 134 - protein, 119 aa, Artificial Sequence
  Synthetic Sequence
EVQLLESGGGLVQPGGSLRLSCAASGFTFNSYAMSWVRQAPGKGLEWVSAISGSGGSTYYADSVKGRFTISRDNSKNTVYLQMNSLRAEDTAVYYCAKKYYVGPADYWGQGTLVTVSSG

SEQ ID NO: 135 - protein, 119 aa, Artificial Sequence
  Synthetic Sequence
EVQLLESGGGLVQPGGSLRLSCAASGFTFNSYAMSWVRQAPGKGLEWVSVISGSGGSTYYADSVKGRFTISRDNSKNTLYLQMNSLRAEDTAVYYCAKKYYVGPADYWGQGTLVTVSSG

SEQ ID NO: 136 - protein, 119 aa, Artificial Sequence
  Synthetic Sequence
EVQLLESGGGLVQPGGSLRLSCAASGFTFNSYAMSWVRQAPGKGLEWVSGISGSGGSTYYADSVKGRFTISRDNSKNTLYLQMNSLRAEDTAVYYCAKKYYVGPADYWGQGTLVTVSSG

SEQ ID NO: 137 - protein, 119 aa, Artificial Sequence
  Synthetic Sequence
EVQVLESGGGLVQPGGSLRLSCAASGFTFNSYAMSWVRQAPGKGLEWVSAISGSGGSTYYADSVKGRFTISRDNSKNTLYLQMNSLRAEDTAVYYCAKKYYVGPADYWGQGTLVTVSSG

SEQ ID NO: 138 - protein, 120 aa, Artificial Sequence
  Synthetic Sequence
EVQLLESGGGLVQPGGSLRLSCAASGFTFNGSYAMSWVRQAPGKGLEWVSAISGSGGSTYYADSVKGRFTISRDNSKNTLYLQMNSLRAEDTAVYYCAKKYYVGPADYWGQGTLVTVSSG

SEQ ID NO: 139 - protein, 119 aa, Artificial Sequence
  Synthetic Sequence
EVQLLESGGGLVQPGGSLRLSCAASGFTFNSYAMNWVRQAPGKGLEWVSAISGSGGSTYYADSVKGRFTISRDNSKNTLYLQMNSLRAEDTAVYYCAKKYYVGPADYWGQGTLVTVSSG

SEQ ID NO: 140 - protein, 119 aa, Artificial Sequence
  Synthetic Sequence
EVQVLESGGGLVQPGGSLRLSCAASGFTFNSYAMSWVRQAPGKGLEWVSGISGSGGSTYYADSVKGRFTISRDNSKNTLYLQMNSLRAEDTAVYYCAKKYYVSPADYWDQGTLVTVSSG

SEQ ID NO: 141 - protein, 120 aa, Artificial Sequence
  Synthetic Sequence
EVQVLESGGGLVQPGGSLRLSCAASGFTFNGSYAMSWVRQAPGKGLEWVSGISGSGGSTYYADSVKGRFTISRDNSKNTLYLQMNSLRAEDTAVYYCAKKYYVSPADYWDQGTLVTVSSG

SEQ ID NO: 142 - protein, 119 aa, Artificial Sequence
  Synthetic Sequence
EVQLLESGGGLVQPGGSLRLSCAASGFTFNSYAMSWVRQAPGKGLEWVSAISGSGGSTYYADSVKGRFTISRDNSKNTLYLQMNSLRAEDTAVYYCAKKYYVGPADYWDQGTLVTVSSG

SEQ ID NO: 143 - protein, 119 aa, Artificial Sequence
  Synthetic Sequence
EVQLLESGGGLVQPGGSLRLSCAASGFTFNSYAMSWVRQAPGKGLEWVSAISGSGGSTYYADSVKGRFTISRDNSKNTLYLQMNSLRAEDTAVYYCAKKYYVSPADYWGQGTLVTVSSG

SEQ ID NO: 144 - protein, 119 aa, Artificial Sequence
  Synthetic Sequence
EVQLLESGGGLVQPGGSLRLSCAASGFTFNSYAMSWVRQAPGKGLEWVSAISGSGGSTYYADSVKGQFTISRDNSKNTLYLQMNSLRAEDTAVYYCAKKYYVGPADYWGQGTLVTVSSG

SEQ ID NO: 145 - protein, 119 aa, Artificial Sequence
  Synthetic Sequence
EVQLLESGGGLVQPGGSLRLSCAASGFTFSSYAMSWVRQAPGKGLEWVSAISGSGGSTYYADSVKGRFTISRDNSKNTLYLQMNSLRAEDTAVYYCAKKYYVGPADYWDQGTLVTVSSG

SEQ ID NO: 146 - protein, 119 aa, Artificial Sequence
  Synthetic Sequence
EVQVLESGGGLVQPGGSLRLSCAASGFTFSSYAMSWVRQAPGKGLEWVSAISGSGGSTYYADSVKGRFTISRDNSKNTLYLQMNSLRAEDTAVYYCAKKYYVGPADYWDQGTLVTVSSG

SEQ ID NO: 147 - protein, 119 aa, Artificial Sequence
  Synthetic Sequence
EVQVLESGGGLVQPGGSLRLSCAASGFTFSSYAMSWVRQAPGKGLEWVSAISGSGGSTYYADSVKGRFTISRDNSKNTLYLQMNSLRAEDTAVYYCAKKYYVGPADYWGQGTLVTVSSG

SEQ ID NO: 148 - protein, 120 aa, Artificial Sequence
  Synthetic Sequence
EVQLLESGGGLVQPGGSLRLSCAASGFTFSGSYAMSWVRQAPGKGLEWVSAISGSGGSTYYADSVKGRFTISRDNSKNTLYLQMNSLRAEDTAVYYCAKKYYVGPADYWDQGTLVTVSSG

SEQ ID NO: 149 - protein, 120 aa, Artificial Sequence
  Synthetic Sequence
EVQVLESGGGLVQPGGSLRLSCAASGFTFSGSYAMSWVRQAPGKGLEWVSAISGSGGSTYYADSVKGRFTISRDNSKNTLYLQMNSLRAEDTAVYYCAKKYYVGPADYWDQGTLVTVSSG

SEQ ID NO: 150 - protein, 120 aa, Artificial Sequence
  Synthetic Sequence
EVQVLESGGGLVQPGGSLRLSCAASGFTFSGSYAMSWVRQAPGKGLEWVSAISGSGGSTYYADSVKGRFTISRDNSKNTLYLQMNSLRAEDTAVYYCAKKYYVGPADYWGQGTLVTVSSG

SEQ ID NO: 151 - protein, 119 aa, Artificial Sequence
  Synthetic Sequence
EVQLLESGGGLVQPGGSLRLSCAASGFTFSSYAMSWVRQAPGKGLEWVSAISGSGGSTYYADSVKGRFTISRDNSKNTLYLQMNSLRAEDTAVYYCAKKYYVSPADYWGQGTLVTVSSG

SEQ ID NO: 152 - protein, 119 aa, Artificial Sequence
  Synthetic Sequence
EVQLLESGGGLVQPGGSLRLSCAASGFTFSSYAMSWVRQAPGKGLEWVSAISGSGGSTYYADSVKGRFTISRDNSKNTLYLQMNSLRAEDTAVYYCAKKYYGSPADYWGQGTLVTVSSG

SEQ ID NO: 153 - protein, 120 aa, Artificial Sequence
  Synthetic Sequence
EVQLLESGGGLVQPGGSLRLSCAASGFTFSGSYAMSWVRQAPGKGLEWVSAISGSGGSTYYADSVKGRFTISRDNSKNTLYLQMNSLRAEDTAVYYCAKKYYDGPADYWDQGTLVTVSSG

SEQ ID NO: 154 - protein, 119 aa, Artificial Sequence
  Synthetic Sequence
EVQLLESGGGLVQPGGSLRLSCAASGFTFNSYAMSWVRQAPGKGLEWVSAISGSGGSTYYVDSVKGRFTISRDNSKNTLYLQMNSLRAEDTAVYYCAKKYYVGPADYWGQGTLVTVSSG

SEQ ID NO: 155 - protein, 119 aa, Artificial Sequence
  Synthetic Sequence
EVQLLESGGGLVQPGGSLRLSCAASGFTFSSYAMSWVRQAPGKGLEWVSAISGSGGSTYYVDSVKGRFTISRDNSKNTLYLQMNSLRAEDTAVYYCAKKYYVSPADYWGQGTLVTVSSG

SEQ ID NO: 156 - protein, 119 aa, Artificial Sequence
  Synthetic Sequence
EVQLLESGGGLVQPGGSLRLSCAASGFTFSSYAMSWVRQAPGKGLEWVSAISGSGGSTYYVDSVKGRFTISRDNSKNTLYLQMNSLRAEDTAVYYCAKKYYVGPADYWDQGTLVTVSSG

SEQ ID NO: 157 - protein, 119 aa, Artificial Sequence
  Synthetic Sequence
EVQLLESGGGLVQPGGSLRLSCAASGFTFSSYAMSWVRQAPGKGLEWVSGISGSGGSTYYVDSVKGRFTISRDNSKNTLYLQMNSLRAEDTAVYYCAKKYYVGPADYWGQGTLVTVSSG

SEQ ID NO: 158 - protein, 119 aa, Artificial Sequence
  Synthetic Sequence
EVQVLESGGGLVQPGGSLRLSCAASGFTFSSYAMSWVRQAPGKGLEWVSAISGSGGSTYYVDSVKGRFTISRDNSKNTLYLQMNSLRAEDTAVYYCAKKYYVGPADYWGQGTLVTVSSG

SEQ ID NO: 159 - protein, 119 aa, Artificial Sequence
  Synthetic Sequence
EVQLLESGGGLIQPGGSLRLSCAASGFTFNSYAMSWVRQAPGKGLEWVSAISGSGGSTYYADSVKGRFTISRDNSKNTLYLQMNSLRAEDTAVYYCAKKYYVGPADYWGQGTLVTVSSG

SEQ ID NO: 160 - protein, 119 aa, Artificial Sequence
  Synthetic Sequence
EVQLLESGGGLIQPGGSLRLSCAASGFTFSSYAMSWVRQAPGKGLEWVSAISGSGGSTYYADSVKGRFTISRDNSKNTLYLQMNSLRAEDTAVYYCAKKYYVSPADYWGQGTLVTVSSG

SEQ ID NO: 161 - protein, 119 aa, Artificial Sequence
  Synthetic Sequence
EVQLLESGGGLIQPGGSLRLSCAASGFTFSSYAMSWVRQAPGKGLEWVSAISGSGGSTYYADSVKGRFTISRDNSKNTLYLQMNSLRAEDTAVYYCAKKYYVGPADYWDQGTLVTVSSG

SEQ ID NO: 162 - protein, 119 aa, Artificial Sequence
  Synthetic Sequence
EVQLLESGGGLIQPGGSLRLSCAASGFTFSSYAMSWVRQAPGKGLEWVSGISGSGGSTYYADSVKGRFTISRDNSKNTLYLQMNSLRAEDTAVYYCAKKYYVGPADYWGQGTLVTVSSG

SEQ ID NO: 163 - protein, 119 aa, Artificial Sequence
  Synthetic Sequence
EVQVLESGGGLIQPGGSLRLSCAASGFTFSSYAMSWVRQAPGKGLEWVSAISGSGGSTYYADSVKGRFTISRDNSKNTLYLQMNSLRAEDTAVYYCAKKYYVGPADYWGQGTLVTVSSG

SEQ ID NO: 164 - protein, 119 aa, Artificial Sequence
  Synthetic Sequence
EVQLLESGGGLVQPGGSLRLSCAASGFTFNSYAMSWVRQAPGKGLEWVSAISGSGGSTYYADSVKGRFTISRDNSKNTVYLQMNSLRAEDTAVYYCAKKYYVSPADYWGQGTLVTVSSG

SEQ ID NO: 165 - protein, 120 aa, Artificial Sequence
  Synthetic Sequence
EVQLLESGGGLVQPGGSLRLSCAASGFTFNGSYAMSWVRQAPGKGLEWVSAISGSGGSTYYADSVKGRFTISRDNSKNTVYLQMNSLRAEDTAVYYCAKKYYVGPADYWGQGTLVTVSSG

SEQ ID NO: 166 - protein, 119 aa, Artificial Sequence
  Synthetic Sequence
EVQLLESGGGLVQPGGSLRLSCAASGFTFNSYAMNWVRQAPGKGLEWVSAISGSGGSTYYADSVKGRFTISRDNSKNTVYLQMNSLRAEDTAVYYCAKKYYVGPADYWGQGTLVTVSSG

SEQ ID NO: 167 - protein, 120 aa, Artificial Sequence
  Synthetic Sequence
EVQVLESGGGLVQPGGSLRLSCAASGFTFNGSYAMSWVRQAPGKGLEWVSGISGSGGSTYYADSVKGRFTISRDNSKNTLYLQMNSLRAEDTAVYYCAKKYYVGPADYWDQGTLVTVSSG

SEQ ID NO: 168 - protein, 120 aa, Artificial Sequence
  Synthetic Sequence
EVQVLESGGGLVQPGGSLRLSCAASGFTFNGSYAMSWVRQAPGKGLEWVSGISGSGGSTYYADSVKGRFTISRDNSKNTLYLQMNSLRAEDTAVYYCAKKYYVSPADYWGQGTLVTVSSG

SEQ ID NO: 169 - protein, 119 aa, Artificial Sequence
  Synthetic Sequence
EVQVLESGGGLVQPGGSLRLSCAASGFTFNSYAMSWVRQAPGKGLEWVSGISGSGGSTYYADSVKGRFTISRDNSKNTLYLQMNSLRAEDTAVYYCAKKYYVGPADYWGQGTLVTVSSG

SEQ ID NO: 170 - protein, 119 aa, Artificial Sequence
  Synthetic Sequence
EVQLLESGGGLVQPGGSLRLSCAASGFTFNSYAMSWVRQAPGKGLEWVSGISGSGGSTYYADSVKGRFTISRDNSKNTVYLQMNSLRAEDTAVYYCAKKYYVGPADYWGQGTLVTVSSG

SEQ ID NO: 171 - protein, 119 aa, Artificial Sequence
  Synthetic Sequence
EVQVLESGGGLVQPGGSLRLSCAASGFTFNSYAMSWVRQAPGKGLEWVSAISGSGGSTYYADSVKGRFTISRDNSKNTLYLQMNSLRAEDTAVYYCAKKYYVGPADYWDQGTLVTVSSG

SEQ ID NO: 172 - protein, 119 aa, Artificial Sequence
  Synthetic Sequence
EVQVLESGGGLVQPGGSLRLSCAASGFTFNSYAMSWVRQAPGKGLEWVSAISGSGGSTYYADSVKGRFTISRDNSKNTLYLQMNSLRAEDTAVYYCAKKYYVSPADYWGQGTLVTVSSG

SEQ ID NO: 173 - protein, 120 aa, Artificial Sequence
  Synthetic Sequence
EVQVLESGGGLVQPGGSLRLSCAASGFTFNGSYAMSWVRQAPGKGLEWVSAISGSGGSTYYADSVKGRFTISRDNSKNTLYLQMNSLRAEDTAVYYCAKKYYVGPADYWGQGTLVTVSSG

SEQ ID NO: 174 - protein, 119 aa, Artificial Sequence
  Synthetic Sequence
EVQVLESGGGLVQPGGSLRLSCAASGFTFNSYAMNWVRQAPGKGLEWVSAISGSGGSTYYADSVKGRFTISRDNSKNTLYLQMNSLRAEDTAVYYCAKKYYVGPADYWGQGTLVTVSSG

SEQ ID NO: 175 - protein, 119 aa, Artificial Sequence
  Synthetic Sequence
EVQVLESGGGLVQPGGSLRLSCAASGFTFNSYAMSWVRQAPGKGLEWVSAISGSGGSTYYADSVKGRFTISRDNSKNTVYLQMNSLRAEDTAVYYCAKKYYVGPADYWGQGTLVTVSSG

SEQ ID NO: 176 - protein, 119 aa, Artificial Sequence
  Synthetic Sequence
EVQVLESGGGLVQPGGSLRLSCAASGFTFNSYAMSWVRQAPGKGLEWVSGISGSGGSTYYADSVKGRFTISRDNSKNTVYLQMNSLRAEDTAVYYCAKKYYVSPADYWGQGTLVTVSSG

SEQ ID NO: 177 - protein, 120 aa, Artificial Sequence
  Synthetic Sequence
EVQVLESGGGLVQPGGSLRLSCAASGFTFNGSYAMSWVRQAPGKGLEWVSAISGSGGSTYYADSVKGRFTISRDNSKNTVYLQMNSLRAEDTAVYYCAKKYYVSPADYWGQGTLVTVSSG

SEQ ID NO: 178 - protein, 119 aa, Artificial Sequence
  Synthetic Sequence
EVQVLESGGGLVQPGGSLRLSCAASGFTFNSYAMSWVRQAPGKGLEWVSGISGSGGSTYYADSVKGRFTISRDNSKNTVYLQMNSLRAEDTAVYYCAKKYYVGPADYWGQGTLVTVSSG

SEQ ID NO: 179 - protein, 120 aa, Artificial Sequence
  Synthetic Sequence
EVQVLESGGGLVQPGGSLRLSCAASGFTFNGSYAMSWVRQAPGKGLEWVSAISGSGGSTYYADSVKGRFTISRDNSKNTVYLQMNSLRAEDTAVYYCAKKYYVGPADYWGQGTLVTVSSG

SEQ ID NO: 180 - protein, 119 aa, Artificial Sequence
  Synthetic Sequence
EVQVLESGGGLVQPGGSLRLSCAASGFTFNSYAMSWVRQAPGKGLEWVSAISGSGGSTYYADSVKGRFTISRDNSKNTVYLQMNSLRAEDTAVYYCAKKYYVSPADYWGQGTLVTVSSG

SEQ ID NO: 181 - protein, 119 aa, Artificial Sequence
  Synthetic Sequence
EVQVLESGGGLVQPGGSLRLSCAASGFTFRSYAMSWVRQAPGKGLEWVSAISGSGGSTYYADSVKGRFTISRDNSKNTLYLQMNSLRAEDTAVYYCAKKYYVGPADYWGQGTLVTVSSG

SEQ ID NO: 182 - protein, 119 aa, Artificial Sequence
  Synthetic Sequence
EVQVLESGGGLVQPGGSLRLSCAASGFTFTSYAMSWVRQAPGKGLEWVSAISGSGGSTYYADSVKGRFTISRDNSKNTLYLQMNSLRAEDTAVYYCAKKYYVGPADYWGQGTLVTVSSG

SEQ ID NO: 183 - protein, 119 aa, Artificial Sequence
  Synthetic Sequence
EVQVLESGGGLVQPGGSLRLSCAASGFTFDSYAMSWVRQAPGKGLEWVSAISGSGGSTYYADSVKGRFTISRDNSKNTLYLQMNSLRAEDTAVYYCAKKYYVGPADYWGQGTLVTVSSG

SEQ ID NO: 184 - protein, 119 aa, Artificial Sequence
  Synthetic Sequence
EVQVLESGGGLVQPGGSLRLSCAASGFTFGSYAMSWVRQAPGKGLEWVSAISGSGGSTYYADSVKGRFTISRDNSKNTLYLQMNSLRAEDTAVYYCAKKYYVGPADYWGQGTLVTVSSG

SEQ ID NO: 185 - protein, 119 aa, Artificial Sequence
  Synthetic Sequence
EVQVLESGGGLVQPGGSLRLSCAASGFTFNSYAMSWVRQAPGKGLEWVSAISGSGGSTYYADSVKGRFTISRDNSKNTTYLQMNSLRAEDTAVYYCAKKYYVGPADYWGQGTLVTVSSG

SEQ ID NO: 186 - protein, 119 aa, Artificial Sequence
  Synthetic Sequence
EVQVLESGGGLVQPGGSLRLSCAASGFTFNSYAMSWVRQAPGKGLEWVSAISGSGGSTYYADSVKGRFTISRDNSKNTMYLQMNSLRAEDTAVYYCAKKYYVGPADYWGQGTLVTVSSG

SEQ ID NO: 187 - protein, 119 aa, Artificial Sequence
  Synthetic Sequence
EVQVLESGGGLVQPGGSLRLSCAASGFTFNSYAMSWVRQAPGKGLEWVSAISGSGGSTYYADSVKGRFTISRDNSKNTPYLQMNSLRAEDTAVYYCAKKYYVGPADYWGQGTLVTVSSG

SEQ ID NO: 188 - protein, 119 aa, Artificial Sequence
  Synthetic Sequence
EVQVLESGGGLVQPGGSLRLSCAASGFTFNSYAMSWVRQAPGKGLEWVSSISGSGGSTYYADSVKGRFTISRDNSKNTLYLQMNSLRAEDTAVYYCAKKYYVGPADYWGQGTLVTVSSG

SEQ ID NO: 189 - protein, 119 aa, Artificial Sequence
  Synthetic Sequence
EVQVLESGGGLVQPGGSLRLSCAASGFTFNSYAMSWVRQAPGKGLEWVSFISGSGGSTYYADSVKGRFTISRDNSKNTLYLQMNSLRAEDTAVYYCAKKYYVGPADYWGQGTLVTVSSG

SEQ ID NO: 190 - protein, 119 aa, Artificial Sequence
  Synthetic Sequence
EVQVLESGGGLVQPGGSLRLSCAASGFTFNSYAMSWVRQAPGKGLEWVSVISGSGGSTYYADSVKGRFTISRDNSKNTLYLQMNSLRAEDTAVYYCAKKYYVGPADYWGQGTLVTVSSG

SEQ ID NO: 191 - protein, 119 aa, Artificial Sequence
  Synthetic Sequence
EVQVLESGGGLVQPGGSLRLSCAASGFTFNSYAMSWVRQAPGKGLEWVSIISGSGGSTYYADSVKGRFTISRDNSKNTLYLQMNSLRAEDTAVYYCAKKYYVGPADYWGQGTLVTVSSG

SEQ ID NO: 192 - protein, 119 aa, Artificial Sequence
  Synthetic Sequence
EVQVLESGGGLVQPGGSLRLSCAASGFTFNSYAMSWVRQAPGKGLEWVSTISGSGGSTYYADSVKGRFTISRDNSKNTLYLQMNSLRAEDTAVYYCAKKYYVGPADYWGQGTLVTVSSG

SEQ ID NO: 193 - protein, 119 aa, Artificial Sequence
  Synthetic Sequence
EVQVLESGGGLVQPGGSLRLSCAASGFTFNSYAMSWVRQAPGKGLEWVSDISGSGGSTYYADSVKGRFTISRDNSKNTLYLQMNSLRAEDTAVYYCAKKYYVGPADYWGQGTLVTVSSG

SEQ ID NO: 194 - protein, 119 aa, Artificial Sequence
  Synthetic Sequence
EVQVLESGGGLVQPGGSLRLSCAASGFTFNSYAMSWVRQAPGKGLEWVSAISGSGGSTYYADSVKGRFTISRDNSKNTLYLQMNSLRAEDTAVYYCAKKYYAGPADYWGQGTLVTVSSG

SEQ ID NO: 195 - protein, 119 aa, Artificial Sequence
  Synthetic Sequence
EVQVLESGGGLVQPGGSLRLSCAASGFTFNSYAMSWVRQAPGKGLEWVSAISGSGGSTYYADSVKGRFTISRDNSKNTLYLQMNSLRAEDTAVYYCAKKYYTGPADYWGQGTLVTVSSG

SEQ ID NO: 196 - protein, 119 aa, Artificial Sequence
  Synthetic Sequence
EVQVLESGGGLVQPGGSLRLSCAASGFTFNSYAMSWVRQAPGKGLEWVSAISGSGGSTYYADSVKGRFTISRDNSKNTLYLQMNSLRAEDTAVYYCAKKYYNGPADYWGQGTLVTVSSG

SEQ ID NO: 197 - protein, 119 aa, Artificial Sequence
  Synthetic Sequence
EVQVLESGGGLVQPGGSLRLSCAASGFTFNSYAMSWVRQAPGKGLEWVSAISGSGGSTYYADSVKGRFTISRDNSKNTLYLQMNSLRAEDTAVYYCAKKYYVVPADYWGQGTLVTVSSG

SEQ ID NO: 198 - protein, 119 aa, Artificial Sequence
  Synthetic Sequence
EVQVLESGGGLVQPGGSLRLSCAASGFTFNSYAMSWVRQAPGKGLEWVSAISGSGGSTYYADSVKGRFTISRDNSKNTLYLQMNSLRAEDTAVYYCAKKYYVDPADYWGQGTLVTVSSG

SEQ ID NO: 199 - protein, 119 aa, Artificial Sequence
  Synthetic Sequence
EVQVLESGGGLVQPGGSLRLSCAASGFTFNSYAMSWVRQAPGKGLEWVSAISGSGGSTYYADSVKGRFTISRDNSKNTLYLQMNSLRAEDTAVYYCAKKYYVNPADYWGQGTLVTVSSG

SEQ ID NO: 200 - protein, 119 aa, Artificial Sequence
  Synthetic Sequence
EVQVLESGGGLVQPGGSLRLSCAASGFTFNSYAMSWVRQAPGKGLEWVSAISGSGGSTYYADSVKGRFTISRDNSKNTLYLQMNSLRAEDTAVYYCAKKYYVTPADYWGQGTLVTVSSG

SEQ ID NO: 201 - protein, 120 aa, Artificial Sequence
  Synthetic Sequence
EVQVLESGGGLVQPGGSLRLSCAASGFTFNGSYAMSWVRQAPGKGLEWVSGISGSGGSTYYADSVKGRFTISRDNSKNTVYLQMNSLRAEDTAVYYCAKKYYVGPADYWGQGTLVTVSSG

SEQ ID NO: 202 - protein, 119 aa, Artificial Sequence
  Synthetic Sequence
EVQMLESGGGLVQPGGSLRLSCAASGFTFNSYAMSWVRQAPGKGLEWVSAISGSGGSTYYADSVKGRFTISRDNSKNTVYLQMNSLRAEDTAVYYCAKKYYVSPADYWGQGTLVTVSSG

SEQ ID NO: 203 - protein, 119 aa, Artificial Sequence
  Synthetic Sequence
EVQMLESGGGLVQPGGSLRLSCAASGFTFNSYAMSWVRQAPGKGLEWVSGISGSGGSTYYADSVKGRFTISRDNSKNTVYLQMNSLRAEDTAVYYCAKKYYVGPADYWGQGTLVTVSSG

SEQ ID NO: 204 - protein, 120 aa, Artificial Sequence
  Synthetic Sequence
EVQVLESGGGLVQPGGSLRLSCAASGFTFSGSYAMSWVRQAPGKGLEWVSGISGSGGSTYYADSVKGRFTISRDNSKNTLYLQMNSLRAEDTAVYYCAKKYYVGPADYWGQGTLVTVSSG

SEQ ID NO: 205 - protein, 120 aa, Artificial Sequence
  Synthetic Sequence
EVQLLESGGGLVQPGGSLRLSCAASGFTFSGSYAMSWVRQAPGKGLEWVSAISGSGGSTYYADSVKGRFTISRDNSKNTVYLQMNSLRAEDTAVYYCAKKYYVGPADYWGQGTLVTVSSG

SEQ ID NO: 206 - protein, 120 aa, Artificial Sequence
  Synthetic Sequence
EVQLLESGGGLVQPGGSLRLSCAASGFTFSGSYAMSWVRQAPGKGLEWVSGISGSGGSTYYADSVKGRFTISRDNSKNTVYLQMNSLRAEDTAVYYCAKKYYVGPADYWGQGTLVTVSSG

SEQ ID NO: 207 - protein, 119 aa, Artificial Sequence
  Synthetic Sequence
EVQVLESGGGLVQPGGSLRLSCAASGFTFNSYAMSWVRQAPGKGLEWVSGISGSGGSTYYADSVKGQFTISRDNSKNTLYLQMNSLRAEDTAVYYCAKKYYVGPADYWGQGTLVTVSSG

SEQ ID NO: 208 - protein, 119 aa, Artificial Sequence
  Synthetic Sequence
EVQLLESGGGLVQPGGSLRLSCAASGFTFNSYAMSWVRQAPGKGLEWVSGISGSGGSTYYADSVKGQFTISRDNSKNTVYLQMNSLRAEDTAVYYCAKKYYVGPADYWGQGTLVTVSSG

SEQ ID NO: 209 - protein, 119 aa, Artificial Sequence
  Synthetic Sequence
EVQVLESGGGLVQPGGSLRLSCAASGFTFNSYAMSWVRQAPGKGLEWVSGISGSGGSTYYADSVKGRFTISRDNSKNTLYLQMNSLRAEDTAVYYCAKKYYDGPADYWGQGTLVTVSSG

SEQ ID NO: 210 - protein, 119 aa, Artificial Sequence
  Synthetic Sequence
EVQLLESGGGLVQPGGSLRLSCAASGFTFNSYAMSWVRQAPGKGLEWVSGISGSGGSTYYADSVKGRFTISRDNSKNTVYLQMNSLRAEDTAVYYCAKKYYDGPADYWGQGTLVTVSSG

SEQ ID NO: 211 - protein, 120 aa, Artificial Sequence
  Synthetic Sequence
EVQVLESGGGLVQPGGSLRLSCAASGFTFSGSYAMSWVRQAPGKGLEWVSGISGSGGSTYYADSVKGRFTISRDNSKNTLYLQMNSLRAEDTAVYYCAKKYYDGPADYWGQGTLVTVSSG

SEQ ID NO: 212 - protein, 120 aa, Artificial Sequence
  Synthetic Sequence
EVQLLESGGGLVQPGGSLRLSCAASGFTFSGSYAMSWVRQAPGKGLEWVSGISGSGGSTYYADSVKGRFTISRDNSKNTVYLQMNSLRAEDTAVYYCAKKYYDGPADYWGQGTLVTVSSG

SEQ ID NO: 213 - protein, 119 aa, Artificial Sequence
  Synthetic Sequence
EVQMLESGGGLVQPGGSLRLSCAASGFTFNSYAMSWVRQAPGKGLEWVSGISGSGGSTYYADSVKGRFTISRDNSKNTLYLQMNSLRAEDTAVYYCAKKYYVGPADYWGQGTLVTVSSG

SEQ ID NO: 214 - protein, 120 aa, Artificial Sequence
  Synthetic Sequence
EVQMLESGGGLVQPGGSLRLSCAASGFTFSGSYAMSWVRQAPGKGLEWVSGISGSGGSTYYADSVKGRFTISRDNSKNTLYLQMNSLRAEDTAVYYCAKKYYVGPADYWGQGTLVTVSSG

SEQ ID NO: 215 - protein, 120 aa, Artificial Sequence
  Synthetic Sequence
EVQMLESGGGLVQPGGSLRLSCAASGFTFSGSYAMSWVRQAPGKGLEWVSGISGSGGSTYYADSVKGRFTISRDNSKNTLYLQMNSLRAEDTAVYYCAKKYYDGPADYWGQGTLVTVSSG

SEQ ID NO: 216 - protein, 120 aa, Artificial Sequence
  Synthetic Sequence
EVQMLESGGGLVQPGGSLRLSCAASGFTFSGSYAMSWVRQAPGKGLEWVSGISGSGGSTYYADSVKGRFTISRDNSKNTVYLQMNSLRAEDTAVYYCAKKYYVGPADYWGQGTLVTVSSG

SEQ ID NO: 217 - protein, 119 aa, Artificial Sequence
  Synthetic Sequence
EVQLLESGGGLVQPGGSLRLSCVASGFTFNSYAMSWVRQAPGKGLEWVSGISGSGGSTYYADSVKGRFTISRDNSKNTVYLQMNSLRAEDTAVYYCAKKYYVGPADYWGQGTLVTVSSG

SEQ ID NO: 218 - protein, 120 aa, Artificial Sequence
  Synthetic Sequence
EVQVLESGGGLVQPGGSLRLSCVASGFTFSGSYAMSWVRQAPGKGLEWVSGISGSGGSTYYADSVKGRFTISRDNSKNTLYLQMNSLRAEDTAVYYCAKKYYVGPADYWGQGTLVTVSSG

SEQ ID NO: 219 - protein, 119 aa, Artificial Sequence
  Synthetic Sequence
EVQMLESGGGLVQPGGSLRLSCAASGFTFNSYAMSWVRQAPGKGLEWVSGISGSGGSTYYADSVKGRFTISRDNSKNTVYLQMNSLRAEDTAVYYCAKKYYDGPADYWGQGTLVTVSSG

SEQ ID NO: 220 - protein, 119 aa, Artificial Sequence
  Synthetic Sequence
EVQLLESGGGLVQPGGSLRLYCAASGFTFNSYAMSWVRQAPGKGLEWVSGISGSGGSTYYADSVKGRFTISRDNSKNTVYLQMNSLRAEDTAVYYCAKKYYVGPADYWGQGTLVTVSSG

SEQ ID NO: 221 - protein, 119 aa, Artificial Sequence
  Synthetic Sequence
EVQLLESGGDLVQPGGSLRLSCAASGFTFNSYAMSWVRQAPGKGLEWVSGISGSGGSTYYADSVKGRFTISRDNSKNTVYLQMNSLRAEDTAVYYCAKKYYVGPADYWGQGTLVTVSSG

SEQ ID NO: 222 - protein, 118 aa, Artificial Sequence
  Synthetic Sequence
EVQLLSGGGLVQPGGSLRLSCAASGFTFNSYAMSWVRQAPGKGLEWVSGISGSGGSTYYADSVKGRFTISRDNSKNTVYLQMNSLRAEDTAVYYCAKKYYVGPADYWGQGTLVTVSSG

SEQ ID NO: 223 - protein, 119 aa, Artificial Sequence
  Synthetic Sequence
EVQLLESGGGLVQPGGSLRLSCAASGFTFNSYAMSWVRQAPGKGLEWVSGISGSGGSTYYADSVKGRFTISRDNSNNTVYLQMNSLRAEDTAVYYCAKKYYVGPADYWGQGTLVTVSSG

SEQ ID NO: 224 - protein, 119 aa, Artificial Sequence
  Synthetic Sequence
EVQLLESGGGLVQPGGSLRLSCAASGFTFNSYAMSWVRQAPGKGLEWVSGISGSGGSTYYVDSVKGRFTISRDNSKNTVYLQMNSLRAEDTAVYYCAKKYYVGPADYWGQGTLVTVSSG

SEQ ID NO: 225 - protein, 119 aa, Artificial Sequence
  Synthetic Sequence
EVQLLESGGGLVQPGGSLRLSCAASGFTFNSYAMSWVRQAPGKGLEWVSGISGSGGNTYYADSVKGRFTISRDNSKNTVYLQMNSLRAEDTAVYYCAKKYYVGPADYWGQGTLVTVSSG

SEQ ID NO: 226 - protein, 120 aa, Artificial Sequence
  Synthetic Sequence
EVQLLESGGGLVQPGGSLRLYCVASGFTFSGSYAMSWVRQAPGKGLEWVSAISGSGGSTYYADSVKGRFTISRDNSKNTLYLQMNSLRAEDTAVYYCAKKYYDGPADYWGQGTLVTVSSG

SEQ ID NO: 227 - protein, 120 aa, Artificial Sequence
  Synthetic Sequence
EVQLLESGGGLVQPGGSLRLYCVASGFTFSGSYAMSWVRQAPGKGLEWVSAISGSGGNTYYADSVKGRFTISRDNSKNTLYLQMNSLRAEDTAVYYCAKKYYDGPADYWGQGTLVTVSSG

SEQ ID NO: 228 - protein, 122 aa, Artificial Sequence
  Synthetic Sequence
EVQLLESLESGGGLVQPGGSLRLSCAASGFTFNSYAMSWVRQAPGKGLEWVSGISGSGGSTYYADSVKGRFTISRDNSKNTVYLQMNSLRAEDTAVYYCAKKYYVGPADYWGQGTLVTVSSG

SEQ ID NO: 229 - protein, 119 aa, Artificial Sequence
  Synthetic Sequence
EVQLLESGGGLVQPGGSLRLYCVASGFTFNSYAMSWVRQAPGKGLEWVSGISGSGGSTYYADSVKGRFTISRDNSKNTVYLQMNSLRAEDTAVYYCAKKYYVGPADYWGQGTLVTVSSG

SEQ ID NO: 230 - protein, 119 aa, Artificial Sequence
  Synthetic Sequence
EVQLLESGGGLVQPGGSLRLYCVASGFTFNSYAMSWVRQAPGKGLEWVSGISGSGGNTYYADSVKGRFTISRDNSKNTVYLQMNSLRAEDTAVYYCAKKYYVGPADYWGQGTLVTVSSG

SEQ ID NO: 231 - protein, 118 aa, Artificial Sequence
  Synthetic Sequence
EVQLLSGGGLVQPGGSLRLYCVASGFTFNSYAMSWVRQAPGKGLEWVSGISGSGGSTYYADSVKGRFTISRDNSKNTVYLQMNSLRAEDTAVYYCAKKYYVGPADYWGQGTLVTVSSG

SEQ ID NO: 232 - protein, 122 aa, Artificial Sequence
  Synthetic Sequence
EVQLLESLESGGGLVQPGGSLRLYCVASGFTFNSYAMSWVRQAPGKGLEWVSGISGSGGSTYYADSVKGRFTISRDNSKNTVYLQMNSLRAEDTAVYYCAKKYYVGPADYWGQGTLVTVSSG

SEQ ID NO: 233 - protein, 119 aa, Artificial Sequence
  Synthetic Sequence
EVQLLESGGDLVQPGGSLRLYCVASGFTFNSYAMSWVRQAPGKGLEWVSGISGSGGSTYYADSVKGRFTISRDNSKNTVYLQMNSLRAEDTAVYYCAKKYYVGPADYWGQGTLVTVSSG

SEQ ID NO: 234 - protein, 120 aa, Artificial Sequence
  Synthetic Sequence
EVQVLESGGDLVQPGGSLRLSCAASGFTFSGSYAMSWVRQAPGKGLEWVSAISGSGGSTYYADSVKGRFTISRDNSKNTLYLQMNSLRAEDTAVYYCAKKYYVGPADYWGQGTLVTVSSG

SEQ ID NO: 235 - protein, 119 aa, Artificial Sequence
  Synthetic Sequence
EVQVLSGGGLVQPGGSLRLSCAASGFTFSGSYAMSWVRQAPGKGLEWVSAISGSGGSTYYADSVKGRFTISRDNSKNTLYLQMNSLRAEDTAVYYCAKKYYVGPADYWGQGTLVTVSSG

SEQ ID NO: 236 - protein, 123 aa, Artificial Sequence
  Synthetic Sequence
EVQVLESLESGGGLVQPGGSLRLSCAASGFTFSGSYAMSWVRQAPGKGLEWVSAISGSGGSTYYADSVKGRFTISRDNSKNTLYLQMNSLRAEDTAVYYCAKKYYVGPADYWGQGTLVTVSSG

SEQ ID NO: 237 - protein, 120 aa, Artificial Sequence
  Synthetic Sequence
EVQVLESGGGLVQPGGSLRLSCVASGFTFSGSYAMSWVRQAPGKGLEWVSAISGSGGSTYYADSVKGRFTISRDNSKNTLYLQMNSLRAEDTAVYYCAKKYYVGPADYWGQGTLVTVSSG

SEQ ID NO: 238 - protein, 120 aa, Artificial Sequence
  Synthetic Sequence
EVQVLESGGGLVQPGGSLRLYCVASGFTFSGSYAMSWVRQAPGKGLEWVSAISGSGGSTYYADSVKGRFTISRDNSKNTLYLQMNSLRAEDTAVYYCAKKYYVGPADYWGQGTLVTVSSG

SEQ ID NO: 239 - protein, 120 aa, Artificial Sequence
  Synthetic Sequence
EVQVLESGGGLVQPGGSLRLYCVASGFTFSGSYAMSWVRQAPGKGLEWVSAISGSGGNTYYADSVKGRFTISRDNSKNTLYLQMNSLRAEDTAVYYCAKKYYVGPADYWGQGTLVTVSSG

SEQ ID NO: 240 - protein, 120 aa, Artificial Sequence
  Synthetic Sequence
EVQLLESGGGLVQPGGSLRLYCVASGFTFSGSYAMSWVRQAPGKGLEWVSAISGSGGNTYYADSVKGRFTISRDNSKNTLYLQMNSLRAEDTAVYYCAKKYYVGPADYWGQGTLVTVSSG

SEQ ID NO: 241 - protein, 120 aa, Artificial Sequence
  Synthetic Sequence
EVQLLESGGGLVQPGGSLRLYCVASGFTFSGSYAMSWVRQAPGKGLEWVSAISGSGGSTYYADSVKGRFTISRDNSKNTLYLQMNSLRAEDTAVYYCAKKYYVGPADYWGQGTLVTVSSG

SEQ ID NO: 242 - protein, 120 aa, Artificial Sequence; identical to SEQ ID NO: 227
  Synthetic Sequence

SEQ ID NO: 243 - protein, 119 aa, Artificial Sequence
  Synthetic Sequence
EVQLLSGGGLVQPGGSLRLYCVASGFTFSGSYAMSWVRQAPGKGLEWVSAISGSGGSTYYADSVKGRFTISRDNSKNTLYLQMNSLRAEDTAVYYCAKKYYDGPADYWGQGTLVTVSSG

SEQ ID NO: 244 - protein, 123 aa, Artificial Sequence
  Synthetic Sequence
EVQLLESLESGGGLVQPGGSLRLYCVASGFTFSGSYAMSWVRQAPGKGLEWVSAISGSGGSTYYADSVKGRFTISRDNSKNTLYLQMNSLRAEDTAVYYCAKKYYDGPADYWGQGTLVTVSSG

SEQ ID NO: 245 - protein, 120 aa, Artificial Sequence
  Synthetic Sequence
EVQLLESGGDLVQPGGSLRLYCVASGFTFSGSYAMSWVRQAPGKGLEWVSAISGSGGSTYYADSVKGRFTISRDNSKNTLYLQMNSLRAEDTAVYYCAKKYYDGPADYWGQGTLVTVSSG

SEQ ID NO: 246 - protein, 120 aa, Artificial Sequence
  Synthetic Sequence
EVQMLESGGGLVQPGGSLRLSCAASGFTFSGSYAMSWVRQAPGKGLEWVSAISGSGGSTYYADSVKGRFTISRDNSKNTLYLQMNSLRAEDTAVYYCAKKYYVGPADYWGQGTLVTVSSG

SEQ ID NO: 247 - protein, 120 aa, Artificial Sequence
  Synthetic Sequence
EVQMLESGGGLVQPGGSLRLYCAASGFTFSGSYAMSWVRQAPGKGLEWVSAISGSGGSTYYADSVKGRFTISRDNSKNTLYLQMNSLRAEDTAVYYCAKKYYVGPADYWGQGTLVTVSSG

SEQ ID NO: 248 - protein, 120 aa, Artificial Sequence
  Synthetic Sequence
EVQMLESGGDLVQPGGSLRLSCAASGFTFSGSYAMSWVRQAPGKGLEWVSAISGSGGSTYYADSVKGRFTISRDNSKNTLYLQMNSLRAEDTAVYYCAKKYYVGPADYWGQGTLVTVSSG

SEQ ID NO: 249 - protein, 120 aa, Artificial Sequence
  Synthetic Sequence
EVQMLESGGGLVQPGGSLRLSCVASGFTFSGSYAMSWVRQAPGKGLEWVSAISGSGGSTYYADSVKGRFTISRDNSKNTLYLQMNSLRAEDTAVYYCAKKYYVGPADYWGQGTLVTVSSG

SEQ ID NO: 250 - protein, 120 aa, Artificial Sequence
  Synthetic Sequence
EVQMLESGGGLVQPGGSLRLYCVASGFTFSGSYAMSWVRQAPGKGLEWVSAISGSGGSTYYADSVKGRFTISRDNSKNTLYLQMNSLRAEDTAVYYCAKKYYVGPADYWGQGTLVTVSSG

SEQ ID NO: 251 - protein, 120 aa, Artificial Sequence
  Synthetic Sequence
EVQMLESGGGLVQPGGSLRLYCVASGFTFSGSYAMSWVRQAPGKGLEWVSAISGSGGNTYYADSVKGRFTISRDNSKNTLYLQMNSLRAEDTAVYYCAKKYYVGPADYWGQGTLVTVSSG

SEQ ID NO: 252 - protein, 120 aa, Artificial Sequence
  Synthetic Sequence
EVQVLESGGGLVQPGGSLRLYCVASGFTFSGSYAMSWVRQAPGKGLEWVSAISGSGGSTYYADSVKGRFTISRDNSKNTLYLQMNSLRAEDTAVYYCAKKYYDGPADYWGQGTLVTVSSG

SEQ ID NO: 253 - protein, 120 aa, Artificial Sequence
  Synthetic Sequence
EVQMLESGGGLVQPGGSLRLYCVASGFTFSGSYAMSWVRQAPGKGLEWVSAISGSGGSTYYADSVKGRFTISRDNSKNTLYLQMNSLRAEDTAVYYCAKKYYDGPADYWGQGTLVTVSSG

SEQ ID NO: 254 - protein, 120 aa, Artificial Sequence
  Synthetic Sequence
EVQVLESGGGLVQPGGSLRLYCAASGFTFSGSYAMSWVRQAPGKGLEWVSAISGSGGSTYYADSVKGRFTISRDNSKNTLYLQMNSLRAEDTAVYYCAKKYYVGPADYWGQGTLVTVSSG

SEQ ID NO: 255 - protein, 120 aa, Artificial Sequence
  Synthetic Sequence
EVQVLESGGGLVQPGGSLRLSCAASGFTFSGSYAMSWVRQAPGKGLEWVSAISGSGGSTYYADSVKGRFTISRDNSKNTLYLQMNNLRAEDTAVYYCAKKYYVGPADYWGQGTLVTVSSG

SEQ ID NO: 256 - protein, 120 aa, Artificial Sequence
  Synthetic Sequence
EVQMLESGGGLVQPGGSLRLSCAASGFTFSGSYAMSWVRQAPGKGLEWVSAISGSGGSTYYADSVKGRFTISRDNSKNTLYLQMNNLRAEDTAVYYCAKKYYVGPADYWGQGTLVTVSSG

SEQ ID NO: 257 - protein, 120 aa, Artificial Sequence
  Synthetic Sequence
EVQVLESGGGLVQPGGSLRLSCAASGFTFSGSYAMSWVRQAPGKGLEWVSAISGSGGSTYYNDSVKGRFTISRDNSKNTLYLQMNSLRAEDTAVYYCAKKYYVGPADYWGQGTLVTVSSG

SEQ ID NO: 258 - protein, 120 aa, Artificial Sequence
  Synthetic Sequence
EVQVLESGGGLVQPGGSLRLYCVASGFTFSGSYVMSWVRQAPGKGLEWVSAISGSGGSTYYADSVKGRFTISRDNSKNTLYLQMNSLRAEDTAVYYCAKKYYVGPADYWGQGTLVTVSSG

SEQ ID NO: 259 - protein, 120 aa, Artificial Sequence
  Synthetic Sequence
EVQVLESGGGLVQPGGSLRLYCVASGFTFSGSYAMSWVRQAPGKGLEWVSAISGSGGSTYYADSVKGRFTISRDNSKNTLYLQMNSLRAEDTAVYYCGKKYYVGPADYWGQGTLVTVSSG

SEQ ID NO: 260 - protein, 113 aa, Artificial Sequence
  Synthetic Sequence
  MISC_FEATURE (40)..(40): Xaa1 is alanine (Ala) or threonine (Thr)
  MISC_FEATURE (43)..(43): Xaa2 is glutamine (Gln) or histidine (His)
  MISC_FEATURE (44)..(44): Xaa3 is glutamine (Gln) or histidine (His)
  MISC_FEATURE (62)..(62): Xaa4 is serine (Ser), tyrosine (Tyr), aspartic acid (Asp), glycine (Gly), threonine (Thr), asparagine (Asn), lysine (Lys), glutamic acid (Glu), leucine (Leu), proline (Pro), or valine (Val)
  MISC_FEATURE (69)..(69): Xaa5 is serine (Ser) or asparagine (Asn)
  MISC_FEATURE (72)..(72): Xaa6 is glycine (Gly), glutamic acid (Glu), alanine (Ala), aspartic acid (Asp), asparagine (Asn), serine (Ser), threonine (Thr), or valine (Val)
  MISC_FEATURE (80)..(80): Xaa7 is threonine (Thr) or isoleucine (Ile)
  MISC_FEATURE (82)..(82): Xaa8 is serine (Ser) or isoleucine (Ile)
  MISC_FEATURE (95)..(95): Xaa9 is glutamine (Gln) or histidine (His)
  MISC_FEATURE (99)..(99): Xaa10 is serine (Ser), asparagine (Asn), arginine (Arg), glycine (Gly), or threonine (Thr)
  MISC_FEATURE (102)..(102): Xaa11 is leucine (Leu) or isoleucine (Ile)
  MISC_FEATURE (112)..(112): Xaa12 is leucine (Leu) or valine (Val)
DIVMTQSPDSLAVSLGERATINCKSSQSVLYSSNNKNYLXWYXXKPGQPPKLLIYWASTREXGVPDRFXGSXSGTDFTLXIXSLQAEDVAVYYCXQYYXSPXTFGGGTKIEXK

SEQ ID NO: 261 - protein, 113 aa, Artificial Sequence
  Synthetic Sequence
DIVMTQSPDSLAVSLGERATINCKSSQSVLYSSNNKNYLAWYQQKPGQPPKLLIYWASTRESGVPDRFSGSGSGTDFTLTISSLQAEDVAVYYCQQYYSSPLTFGGGTKIELK

SEQ ID NO: 262 - protein, 113 aa, Artificial Sequence
  Synthetic Sequence
DIVMTQSPDSLAVSLGERATINCKSSQSVLYSSNNKNYLAWYQQKPGQPPKLLIYWASTRESGVPDRFSGSESGTDFTLTISSLQAEDVAVYYCQQYYSSPLTFGGGTKIELK

SEQ ID NO: 263 - protein, 113 aa, Artificial Sequence
  Synthetic Sequence
DIVMTQSPDSLAVSLGERATINCKSSQSVLYSSNNKNYLAWYQQKPGQPPKLLIYWASTRESGVPDRFSGSESGTDFTLTISSLQAEDVAVYYCQQYYTSPLTFGGGTKIELK

SEQ ID NO: 264 - protein, 113 aa, Artificial Sequence
  Synthetic Sequence
DIVMTQSPDSLAVSLGERATINCKSSQSVLYSSNNKNYLAWYQQKPGQPPKLLIYWASTRESGVPDRFSGSGSGTDFTLTISSLQAEDVAVYYCQQYYNSPLTFGGGTKIELK

SEQ ID NO: 265 - protein, 113 aa, Artificial Sequence
  Synthetic Sequence
DIVMTQSPDSLAVSLGERATINCKSSQSVLYSSNNKNYLAWYQQKPGQPPKLLIYWASTRESGVPDRFSGSGSGTDFTLTISSLQAEDVAVYYCHQYYSSPLTFGGGTKIELK

SEQ ID NO: 266 - protein, 113 aa, Artificial Sequence
  Synthetic Sequence
DIVMTQSPDSLAVSLGERATINCKSSQSVLYSSNNKNYLAWYQQKPGQPPKLLIYWASTRESGVPDRFSGSESGTDFTLTISSLQAEDVAVYYCQQYYNSPLTFGGGTKIELK

SEQ ID NO: 267 - protein, 113 aa, Artificial Sequence
  Synthetic Sequence
DIVMTQSPDSLAVSLGERATINCKSSQSVLYSSNNKNYLAWYQQKPGQPPKLLIYWASTREYGVPDRFSGSESGTDFTLTISSLQAEDVAVYYCQQYYSSPLTFGGGTKIELK

SEQ ID NO: 268 - protein, 113 aa, Artificial Sequence
  Synthetic Sequence
DIVMTQSPDSLAVSLGERATINCKSSQSVLYSSNNKNYLAWYHQKPGQPPKLLIYWASTRESGVPDRFSGSESGTDFTLTISSLQAEDVAVYYCQQYYSSPLTFGGGTKIELK

SEQ ID NO: 269 - protein, 113 aa, Artificial Sequence
  Synthetic Sequence
DIVMTQSPDSLAVSLGERATINCKSSQSVLYSSNNKNYLAWYQQKPGQPPKLLIYWASTRESGVPDRFSGSESGTDFTLIISSLQAEDVAVYYCQQYYSSPLTFGGGTKIELK

SEQ ID NO: 270 - protein, 113 aa, Artificial Sequence
  Synthetic Sequence
DIVMTQSPDSLAVSLGERATINCKSSQSVLYSSNNKNYLAWYQQKPGQPPKLLIYWASTRESGVPDRFSGSESGTDFTLTISSLQAEDVAVYYCQQYYSSPLTFGGGTKIEVK

SEQ ID NO: 271 - protein, 113 aa, Artificial Sequence
  Synthetic Sequence
DIVMTQSPDSLAVSLGERATINCKSSQSVLYSSNNKNYLAWYQQKPGQPPKLLIYWASTRESGVPDRFSGSESGTDFTLTIISLQAEDVAVYYCQQYYSSPLTFGGGTKIELK

SEQ ID NO: 272 - protein, 113 aa, Artificial Sequence
  Synthetic Sequence
DIVMTQSPDSLAVSLGERATINCKSSQSVLYSSNNKNYLAWYQQKPGQPPKLLIYWASTRESGVPDRFNGSESGTDFTLTISSLQAEDVAVYYCQQYYSSPLTFGGGTKIELK

SEQ ID NO: 273 - protein, 113 aa, Artificial Sequence
  Synthetic Sequence
DIVMTQSPDSLAVSLGERATINCKSSQSVLYSSNNKNYLTWYQQKPGQPPKLLIYWASTRESGVPDRFSGSESGTDFTLTISSLQAEDVAVYYCQQYYSSPLTFGGGTKIELK

SEQ ID NO: 274 - protein, 113 aa, Artificial Sequence
  Synthetic Sequence
DIVMTQSPDSLAVSLGERATINCKSSQSVLYSSNNKNYLAWYQQKPGQPPKLLIYWASTRESGVPDRFSGSESGTDFTLTIISLQAEDVAVYYCQQYYNSPLTFGGGTKIELK

SEQ ID NO: 275 - protein, 113 aa, Artificial Sequence
  Synthetic Sequence
DIVMTQSPDSLAVSLGERATINCKSSQSVLYSSNNKNYLAWYQQKPGQPPKLLIYWASTRESGVPDRFNGSESGTDFTLTISSLQAEDVAVYYCQQYYNSPLTFGGGTKIELK

SEQ ID NO: 276 - protein, 113 aa, Artificial Sequence
  Synthetic Sequence
DIVMTQSPDSLAVSLGERATINCKSSQSVLYSSNNKNYLTWYQQKPGQPPKLLIYWASTRESGVPDRFSGSESGTDFTLTISSLQAEDVAVYYCQQYYNSPLTFGGGTKIELK

SEQ ID NO: 277 - protein, 113 aa, Artificial Sequence
  Synthetic Sequence
DIVMTQSPDSLAVSLGERATINCKSSQSVLYSSNNKNYLAWYQQKPGQPPKLLIYWASTREYGVPDRFSGSESGTDFTLTISSLQAEDVAVYYCQQYYRSPLTFGGGTKIELK

SEQ ID NO: 278 - protein, 113 aa, Artificial Sequence
  Synthetic Sequence
DIVMTQSPDSLAVSLGERATINCKSSQSVLYSSNNKNYLAWYQQKPGQPPKLLIYWASTREYGVPDRFSGSESGTDFTLTISSLQAEDVAVYYCQQYYNSPLTFGGGTKIELK

SEQ ID NO: 279 - protein, 113 aa, Artificial Sequence
  Synthetic Sequence
DIVMTQSPDSLAVSLGERATINCKSSQSVLYSSNNKNYLAWYQQKPGQPPKLLIYWASTREDGVPDRFSGSESGTDFTLTISSLQAEDVAVYYCQQYYRSPLTFGGGTKIELK

SEQ ID NO: 280 - protein, 113 aa, Artificial Sequence
  Synthetic Sequence
DIVMTQSPDSLAVSLGERATINCKSSQSVLYSSNNKNYLAWYQQKPGQPPKLLIYWASTREGGVPDRFSGSESGTDFTLTISSLQAEDVAVYYCQQYYRSPLTFGGGTKIELK

SEQ ID NO: 281 - protein, 113 aa, Artificial Sequence
  Synthetic Sequence
DIVMTQSPDSLAVSLGERATINCKSSQSVLYSSNNKNYLAWYQQKPGQPPKLLIYWASTRETGVPDRFSGSESGTDFTLTISSLQAEDVAVYYCQQYYRSPLTFGGGTKIELK

SEQ ID NO: 282 - protein, 113 aa, Artificial Sequence
  Synthetic Sequence
DIVMTQSPDSLAVSLGERATINCKSSQSVLYSSNNKNYLAWYQQKPGQPPKLLIYWASTRENGVPDRFSGSESGTDFTLTISSLQAEDVAVYYCQQYYRSPLTFGGGTKIELK

SEQ ID NO: 283 - protein, 113 aa, Artificial Sequence
  Synthetic Sequence
DIVMTQSPDSLAVSLGERATINCKSSQSVLYSSNNKNYLAWYQQKPGQPPKLLIYWASTREKGVPDRFSGSESGTDFTLTISSLQAEDVAVYYCQQYYRSPLTFGGGTKIELK

SEQ ID NO: 284 - protein, 113 aa, Artificial Sequence
  Synthetic Sequence
DIVMTQSPDSLAVSLGERATINCKSSQSVLYSSNNKNYLAWYQQKPGQPPKLLIYWASTREEGVPDRFSGSESGTDFTLTISSLQAEDVAVYYCQQYYRSPLTFGGGTKIELK

SEQ ID NO: 285 - protein, 113 aa, Artificial Sequence
  Synthetic Sequence
DIVMTQSPDSLAVSLGERATINCKSSQSVLYSSNNKNYLAWYQQKPGQPPKLLIYWASTRELGVPDRFSGSESGTDFTLTISSLQAEDVAVYYCQQYYRSPLTFGGGTKIELK

SEQ ID NO: 286 - protein, 113 aa, Artificial Sequence
  Synthetic Sequence
DIVMTQSPDSLAVSLGERATINCKSSQSVLYSSNNKNYLAWYQQKPGQPPKLLIYWASTREPGVPDRFSGSESGTDFTLTISSLQAEDVAVYYCQQYYRSPLTFGGGTKIELK

SEQ ID NO: 287 - protein, 113 aa, Artificial Sequence
  Synthetic Sequence
DIVMTQSPDSLAVSLGERATINCKSSQSVLYSSNNKNYLAWYQQKPGQPPKLLIYWASTREVGVPDRFSGSESGTDFTLTISSLQAEDVAVYYCQQYYRSPLTFGGGTKIELK

SEQ ID NO: 288 - protein, 113 aa, Artificial Sequence
  Synthetic Sequence
DIVMTQSPDSLAVSLGERATINCKSSQSVLYSSNNKNYLAWYQQKPGQPPKLLIYWASTREYGVPDRFSGSASGTDFTLTISSLQAEDVAVYYCQQYYRSPLTFGGGTKIELK

SEQ ID NO: 289 - protein, 113 aa, Artificial Sequence
  Synthetic Sequence
DIVMTQSPDSLAVSLGERATINCKSSQSVLYSSNNKNYLAWYQQKPGQPPKLLIYWASTREYGVPDRFSGSDSGTDFTLTISSLQAEDVAVYYCQQYYRSPLTFGGGTKIELK

SEQ ID NO: 290 - protein, 113 aa, Artificial Sequence
  Synthetic Sequence
DIVMTQSPDSLAVSLGERATINCKSSQSVLYSSNNKNYLAWYQQKPGQPPKLLIYWASTREYGVPDRFSGSNSGTDFTLTISSLQAEDVAVYYCQQYYRSPLTFGGGTKIELK

SEQ ID NO: 291 - protein, 113 aa, Artificial Sequence
  Synthetic Sequence
DIVMTQSPDSLAVSLGERATINCKSSQSVLYSSNNKNYLAWYQQKPGQPPKLLIYWASTREYGVPDRFSGSSSGTDFTLTISSLQAEDVAVYYCQQYYRSPLTFGGGTKIELK

SEQ ID NO: 292 - protein, 113 aa, Artificial Sequence
  Synthetic Sequence
DIVMTQSPDSLAVSLGERATINCKSSQSVLYSSNNKNYLAWYQQKPGQPPKLLIYWASTREYGVPDRFSGSTSGTDFTLTISSLQAEDVAVYYCQQYYRSPLTFGGGTKIELK

SEQ ID NO: 293 - protein, 113 aa, Artificial Sequence
  Synthetic Sequence
DIVMTQSPDSLAVSLGERATINCKSSQSVLYSSNNKNYLAWYQQKPGQPPKLLIYWASTREYGVPDRFSGSVSGTDFTLTISSLQAEDVAVYYCQQYYRSPLTFGGGTKIELK

SEQ ID NO: 294 - protein, 113 aa, Artificial Sequence
  Synthetic Sequence
DIVMTQSPDSLAVSLGERATINCKSSQSVLYSSNNKNYLAWYQQKPGQPPKLLIYWASTREYGVPDRFSGSESGTDFTLTISSLQAEDVAVYYCQQYYGSPLTFGGGTKIELK

SEQ ID NO: 295 - protein, 113 aa, Artificial Sequence
  Synthetic Sequence
DIVMTQSPDSLAVSLGERATINCKSSQSVLYSSNNKNYLAWYQQKPGQPPKLLIYWASTREYGVPDRFSGSESGTDFTLTISSLQAEDVAVYYCQQYYTSPLTFGGGTKIELK

SEQ ID NO: 296 - protein, 113 aa, Artificial Sequence
  Synthetic Sequence
DIVMTQSPDSLAVSLGERATINCKSSQSVLYSSNNKNYLAWYQQKPGQPPKLLIYWASTREYGVPDRFSGSESGTDFTLTISSLQAEDVAVYYCHQYYNSPLTFGGGTKIELK

SEQ ID NO: 297 - protein, 113 aa, Artificial Sequence
  Synthetic Sequence
DIVMTQSPDSLAVSLGERATINCKSSQSVLYSSNNKNYLAWYQQKPGQPPKLLIYWASTREYGVPDRFSGSESGTDFTLTIISLQAEDVAVYYCQQYYNSPLTFGGGTKIELK

SEQ ID NO: 298 - protein, 113 aa, Artificial Sequence
  Synthetic Sequence
DIVMTQSPDSLAVSLGERATINCKSSQSVLYSSNNKNYLAWYQQKPGQPPKLLIYWASTREYGVPDRFSGSESGTDFTLTISSLQAEDVAVYYCQQYYNSPLTFGGGTKIEVK

SEQ ID NO: 299 - protein, 113 aa, Artificial Sequence
  Synthetic Sequence
DIVMTQSPDSLAVSLGERATINCKSSQSVLYSSNNKNYLTWYQQKPGQPPKLLIYWASTREYGVPDRFSGSESGTDFTLTISSLQAEDVAVYYCQQYYNSPLTFGGGTKIELK

SEQ ID NO: 300 - protein, 113 aa, Artificial Sequence
  Synthetic Sequence
DIVMTQSPDSLAVSLGERATINCKSSQSVLYSSNNKNYLAWYQQKPGQPPKLLIYWASTREYGVPDRFSGSESGTDFTLIISSLQAEDVAVYYCQQYYNSPLTFGGGTKIELK

SEQ ID NO: 301 - protein, 113 aa, Artificial Sequence
  Synthetic Sequence
DIVMTQSPDSLAVSLGERATINCKSSQSVLYSSNNKNYLAWYQHKPGQPPKLLIYWASTREYGVPDRFSGSESGTDFTLTISSLQAEDVAVYYCQQYYNSPLTFGGGTKIELK

SEQ ID NO: 302 - protein, 113 aa, Artificial Sequence
  Synthetic Sequence
DIVMTQSPDSLAVSLGERATINCKSSQSVLYSSNNKNYLAWYHQKPGQPPKLLIYWASTREYGVPDRFSGSESGTDFTLTISSLQAEDVAVYYCQQYYNSPLTFGGGTKIELK

SEQ ID NO: 303 - protein, 113 aa, Artificial Sequence
  Synthetic Sequence
DIVMTQSPDSLAVSLGERATINCKSSQSVLYSSNNKNYLAWYQQKPGQPPKLLIYWASTREYGVPDRFSGSESGTDFTLTISSLQAEDVAVYYCQQYYSSPLTFGGGTKIEVK

SEQ ID NO: 304 - protein, 113 aa, Artificial Sequence
  Synthetic Sequence
DIVMTQSPDSLAVSLGERATINCKSSQSVLYSSNNKNYLAWYQQKPGQPPKLLIYWASTREYGVPDRFSGSESGTDFTLTISSLQAEDVAVYYCQQYYRSPLTFGGGTKIEVK

SEQ ID NO: 305 - protein, 113 aa, Artificial Sequence
  Synthetic Sequence
DIVMTQSPDSLAVSLGERATINCKSSQSVLYSSNNKNYLAWYQQKPGQPPKLLIYWASTREYGVPDRFSGSESGTDFTLTISSLQAEDVAVYYCHQYYRSPLTFGGGTKIEVK

SEQ ID NO: 306 - protein, 113 aa, Artificial Sequence
  Synthetic Sequence
DIVMTQSPDSLAVSLGERATINCKSSQSVLYSSNNKNYLAWYQQKPGQPPKLLIYWASTREYGVPDRFSGSESGTDFTLIISSLQAEDVAVYYCQQYYSSPLTFGGGTKIELK

SEQ ID NO: 307 - protein, 113 aa, Artificial Sequence
  Synthetic Sequence
DIVMTQSPDSLAVSLGERATINCKSSQSVLYSSNNKNYLAWYQQKPGQPPKLLIYWASTREYGVPDRFSGSESGTDFTLTISSLQAEDVAVYYCHQYYRSPLTFGGGTKIELK

SEQ ID NO: 308 - protein, 113 aa, Artificial Sequence
  Synthetic Sequence
DIVMTQSPDSLAVSLGERATINCKSSQSVLYSSNNKNYLAWYQQKPGQPPKLLIYWASTREYGVPDRFSGSESGTDFTLIISSLQAEDVAVYYCHQYYRSPLTFGGGTKIEVK

SEQ ID NO: 309 - protein, 113 aa, Artificial Sequence
  Synthetic Sequence
DIVMTQSPDSLAVSLGERATINCKSSQSVLYSSNNKNYLAWYQQKPGQPPKLLIYWASTREYGVPDRFSGSESGTDFTLIISSLQAEDVAVYYCQQYYSSPLTFGGGTKIEVK

SEQ ID NO: 310 - protein, 113 aa, Artificial Sequence
  Synthetic Sequence
DIVMTQSPDSLAVSLGERATINCKSSQSVLYSSNNKNYLAWYQQKPGQPPKLLIYWASTREYGVPDRFSGSESGTDFTLTISSLQAEDVAVYYCHQYYSSPLTFGGGTKIEVK

SEQ ID NO: 311 - protein, 113 aa, Artificial Sequence
  Synthetic Sequence
DIVMTQSPDSLAVSLGERATINCKSSQSVLYSSNNKNYLAWYQQKPGQPPKLLIYWASTREYGVPDRFSGSESGTDFTLIISSLQAEDVAVYYCHQYYSSPLTFGGGTKIELK

SEQ ID NO: 312 - protein, 113 aa, Artificial Sequence
  Synthetic Sequence
DIVMTQSPDSLAVSLGERATINCKSSQSVLYSSNNKNYLAWYQQKPGQPPKLLIYWASTREYGVPDRFSGSESGTDFTLIISSLQAEDVAVYYCQQYYRSPLTFGGGTKIELK

SEQ ID NO: 313 - protein, 113 aa, Artificial Sequence; identical to SEQ ID NO: 307
  Synthetic Sequence

SEQ ID NO: 314 - protein, 113 aa, Artificial Sequence
  Synthetic Sequence
DIVMTQSPDSLAVSLGERATINCKSSQSVLYSSNNKNYLAWYQQKPGQPPKLLIYWASTREYGVPDRFSGSESGTDFTLIISSLQAEDVAVYYCHQYYRSPLTFGGGTKIELK

SEQ ID NO: 315 - protein, 113 aa, Artificial Sequence
  Synthetic Sequence
DIVMTQSPDSLAVSLGERATINCKSSQSVLYSSNNKNYLAWYQQKPGQPPKLLIYWASTREYGVPDRFSGSESGTDFTLIISSLQAEDVAVYYCQQYYRSPLTFGGGTKIEVK

SEQ ID NO: 316 - protein, 113 aa, Artificial Sequence
  Synthetic Sequence
DIVMTQSPDSLAVSLGERATINCKSSQSVLYSSNNKNYLAWYQQKPGQPPKLLIYWASTRESGVPDRFSGSGSGTDFTLTISSLQAEDVAVYYCQQYYSSPLTFGGGTKIEVK

SEQ ID NO: 317 - protein, 113 aa, Artificial Sequence
  Synthetic Sequence
DIVMTQSPDSLAVSLGERATINCKSSQSVLYSSNNKNYLAWYQQKPGQPPKLLIYWASTRESGVPDRFSGSGSGTDFTLTISSLQAEDVAVYYCHQYYRSPLTFGGGTKIEVK

SEQ ID NO: 318 - protein, 113 aa, Artificial Sequence
  Synthetic Sequence
DIVMTQSPDSLAVSLGERATINCKSSQSVLYSSNNKNYLAWYQQKPGQPPKLLIYWASTRESGVPDRFSGSGSGTDFTLIISSLQAEDVAVYYCQQYYRSPLTFGGGTKIEVK

SEQ ID NO: 319 - protein, 113 aa, Artificial Sequence
  Synthetic Sequence
DIVMTQSPDSLAVSLGERATINCKSSQSVLYSSNNKNYLAWYQQKPGQPPKLLIYWASTRESGVPDRFSGSGSGTDFTLIISSLQAEDVAVYYCQQYYRSPLTFGGGTKIELK

SEQ ID NO: 320 - protein, 113 aa, Artificial Sequence
  Synthetic Sequence
DIVMTQSPDSLAVSLGERATINCKSSQSVLYSSNNKNYLAWYQQKPGQPPKLLIYWASTRESGVPDRFSGSGSGTDFTLIISSLQAEDVAVYYCHQYYSSPLTFGGGTKIEVK

SEQ ID NO: 321 - protein, 113 aa, Artificial Sequence
  Synthetic Sequence
DIVMTQSPDSLAVSLGERATINCKSSQSVLYSSNNKNYLAWYQQKPGQPPKLLIYWASTRESGVPDRFSGSGSGTDFTLTISSLQAEDVAVYYCHQYYRSPLTFGGGTKIELK

SEQ ID NO: 322 - protein, 113 aa, Artificial Sequence
  Synthetic Sequence
DIVMTQSPDSLAVSLGERATINCKSSQSVLYSSNNKNYLAWYQQKPGQPPKLLIYWASTREYGVPDRFSGSESGTDFTLTISSLQAEDVAVYYCHQYYNSPITFGGGTKIELK

SEQ ID NO: 323 - protein, 113 aa, Artificial Sequence
  Synthetic Sequence
DIVMTQSPDSLAVSLGERATINCKSSQSVLYSSNNKNYLAWYQHKPGQPPKLLIYWASTREYGVPDRFSGSESGTDFTLTISSLQAEDVAVYYCQQYYSSPLTFGGGTKIEVK

SEQ ID NO: 324 - protein, 113 aa, Artificial Sequence
  Synthetic Sequence
DIVMTQSPDSLAVSLGERATINCKSSQSVLYSSNNKNYLAWYQQKPGQPPKLLIYWASTREYGVPDRFSGSESGTDFTLTISSLQAEDVAVYYCQQYYSSPITFGGGTKIEVK

SEQ ID NO: 325 - protein, 113 aa, Artificial Sequence
  Synthetic Sequence
DIVMTQSPDSLAVSLGERATINCKSSQSVLYSSNNKNYLAWYQHKPGQPPKLLIYWASTREYGVPDRFSGSESGTDFTLTISSLQAEDVAVYYCQQYYNSPLTFGGGTKIEVK

SEQ ID NO: 326 - protein, 113 aa, Artificial Sequence
  Synthetic Sequence
DIVMTQSPDSLAVSLGERATINCKSSQSVLYSSNNKNYLAWYQHKPGQPPKLLIYWASTREYGVPDRFSGSESGTDFTLTISSLQAEDVAVYYCQQYYNSPITFGGGTKIEVK

SEQ ID NO: 327 - protein, 113 aa, Artificial Sequence
  Synthetic Sequence
DIVMTQSPDSLAVSLGERATINCKSSQSVLYSSNNKNYLAWYQHKPGQPPKLLIYWASTRESGVPDRFSGSGSGTDFTLTISSLQAEDVAVYYCQQYYSSPLTFGGGTKIEVK

SEQ ID NO: 328 - protein, 113 aa, Artificial Sequence
  Synthetic Sequence
DIVMTQSPDSLAVSLGERATINCKSSQSVLYSSNNKNYLAWYQHKPGQPPKLLIYWASTREYGVPDRFSGSESGTDFTLTISSLQAEDVAVYYCQQYYNSPITFGGGTKIELK

SEQ ID NO: 329 - protein, 10 aa, Artificial Sequence
  Synthetic Sequence
GFTFSSYDMS

SEQ ID NO: 330 - protein, 17 aa, Artificial Sequence
  Synthetic Sequence
TISGGGTYTYYQDSVKG

SEQ ID NO: 331 - protein, 3 aa, Artificial Sequence
  Synthetic Sequence
MDY

SEQ ID NO: 332 - protein, 11 aa, Artificial Sequence
  Synthetic Sequence
RASQSIRRYLN

SEQ ID NO: 333 - protein, 7 aa, Artificial Sequence
  Synthetic Sequence
GASTLQS

SEQ ID NO: 334 - protein, 9 aa, Artificial Sequence
  Synthetic Sequence
QQSHSAPLT

SEQ ID NO: 335 - protein, 11 aa, Artificial Sequence
  Synthetic Sequence
GFTFSGSYAMS

SEQ ID NO: 336 - protein, 17 aa, Artificial Sequence
  Synthetic Sequence
AISGSGGSTYYADSVKG

SEQ ID NO: 337 - protein, 9 aa, Artificial Sequence
  Synthetic Sequence
KYYVGPADY

SEQ ID NO: 338 - protein, 17 aa, Artificial Sequence
  Synthetic Sequence
KSSQSVLYSSNNKNYLA

SEQ ID NO: 339 - protein, 7 aa, Artificial Sequence
  Synthetic Sequence
WASTRES

SEQ ID NO: 340 - protein, 9 aa, Artificial Sequence
  Synthetic Sequence
QQYYSSPLT